European Patent Specification EP 2 853 598 B1, published September 13, 2023. Title: METHODS AND COMPOSITIONS FOR OBTAINING USEFUL PLANT TRAITS. Applicant: Board of Regents of the University of Nebraska. The sequence listing filed with the application follows.

SEQUENCE LISTING (56 sequences)

SEQ ID NO: 1 - DNA, 3730 bp, Arabidopsis thaliana
agaggactgtgagattgtgaattgcatagtcgtcgtcttctggcgggaaaagaagccctagaaaaagggtgaaaggtgaaaactctacttcttcttcttcttcttcttcagagtgtgagagagatgcattggattgctaccagaaacgccgtcgtttcattcccaaaatggcggttcttcttccgctcctcatatcgcacttactcttccctcaaaccctcctccccaattctacttaatagaaggtactctgaggggatatcttgtctcagagatggaaagtctttgaaaagaatcacaacggcttctaagaaagtgaagacgtcaagtgatgttctcactgacaaagatctctctcatttggtttggtggaaggagagattgcagacatgtaagaaaccatctactcttcagcttattgaaaggcttatgtacaccaatttacttggtttggaccctagcttgaggaatggaagtttaaaagatggaaacctcaactgggagatgttgcagtttaagtcaaggtttccacgcgaagttttgctctgcagagtaggagaattttatgaggctattggaatagatgcttgtatacttgttgaatatgctggtctcaatccttttggtggtcttcgatcagatagtattccaaaggctggctgcccaattatgaatcttcgacagactttggatgacctgacacgcaatggttattcagtgtgtattgtggaggaagttcaggggccaacaccagcacgctcccgtaaaggtcgatttatttcagggcatgcacatccaggaagtccttatgtatatgggcttgtcggtgttgaccatgatcttgactttcctgatcctatgcctgttgttgggatatctcgttcagcaagggggtattgtatgatatctattttcgagactatgaaagcatattcgctagatgatggtctaacagaagaagccttagttaccaagctccgcactcgtcgctgtcatcatcttttcttacatgcatcgttgaggcacaatgcatcagggacgtgccgctggggagagtttggggaagggggtctactctggggagaatgcagtagcaggaattttgaatggtttgaaggagatactctttccgagctcttatcaagggtcaaagatgtttatggtcttgatgatgaagtttcctttagaaatgtcaatgtaccttcaaaaaatcggccacgtccgttgcatcttggaacggctacacaaattggtgccttacctactgaaggaataccttgtttgttgaaggtgttacttccatctacgtgcagtggtctgccttctttgtatgttagggatcttcttctgaaccctcctgcttacgatattgctctgaaaattcaagaaacgtgcaagctcatgagcacagtaacatgttcaattccagagtttacctgcgtctcttctgctaagcttgtgaagcttcttgagcaacgggaagccaactacattgagttctgtcgaataaaaaatgtgcttgatgatgtattacatatgcatagacatgctgagcttgtggaaatcctgaaattattgatggatcctacctgggtggctactggtttgaaaattgactttgacacttttgtcaacgaatgtcattgggcgtctgatacaattggtgaaatgatctctttagatgagaatgaaagtcatcagaatgtaagtaaatgtgacaatgtcccgaacgaattcttttatgatatggagtcttcatggcgaggtcgcgttaagggaattcatatagaggaagaaatcactcaagtagaaaaatcagctgaggctttatctttagcagtagctgaggattttcaccctattatatcaagaattaaggccaccactgcttcacttggtggcccgaaaggcgaaatcgcatatgcaagagagcatgagtctgtttggttcaaggggaaacggtttacgccatctatctgggctggtactgcaggggaagaccaaataaaacagctgaaacctgccttagactcgaaaggaaaaaaggttggagaagaatggtttacgaccccaaaggtggaaattgctttagtcagataccatgaagctagtgagaatgcaaaagctcgggtgttggaactgttgcgcgagttatccgttaaattgcaaacaaaaataaatgttcttgtctttgcatctatgcttctggtcatttcaaaagcattattttcccatgcttgtgaagggagaaggcgaaagtgggtttttccaacgcttgtcggattcagtttagatgagggcgcaaaaccattagatggtgccagtcgaatgaagctgacaggcctgtcaccttattggtttgatgtatcttctggaaccgctgttcacaataccgttgacatgcaatcactgtttcttctaactggacctaacggtggtggtaaatcgagtttgctcagatcaatatgcgcagctgctctacttggaatttccggtttaatggttccagctgaatcagcttgtattcctcactttgattccatcatgcttcacatgaaatcatatgacagccctgtagacggaaaaagttctttccaggtagaaatgtcggaaatacgatctattgtaagccaggctacttcgagaagcctagtgcttatagatgagatatgccgagggacagagacagcaaaaggcacctgtatcgctggtagtgtggtagagagtcttgacacaagtggttgtttgggtattgtatctactcatctccatggaatcttcagtttacctcttacagcgaaaaacatcacatataaagcaatgggagccgaaaatgtcgaagggcaaaccaagccaacttggaaattgacagatggagtctgcagagagagtcttgcgtttgaaacagctaagagggaaggtgttcccgagtcagttatccaaagagctgaagctctttacctctcggtctatgcaaaagacgcatcagctgaagttgtcaaacccgaccaaatcataacttcatccaacaatgaccagcagatccaaaaaccagtcagctctgagagaagtttggagaaggacttagcaaaagctatcgtcaaaatctgtgggaaaaagatgattgagcctgaagcaatagaatgtctttcaattggtgctcgtgagcttccacctccatctacagttggttcttcatgcgtgtatgtgatgcggagacccgataagagattgtacattggacagaccgatgatcttgaaggacgaatacgtgcgcatcgagcaaaggaaggactgcaagggtcaagttttctataccttatggttcaaggtaagagcatggcttgtcagttagagactctattgattaatcaactccatgaacaaggctactctctggctaacctagccgatggaaagcaccgtaatttcggaacgtcctcaagcttgagtacatcagacgtagtcagcatcttatagtttgaaacattagctgtgtttgtagttgatcatctctatgtgcaattgaacaagtcagtttgctagaactagagtagattactaagaaaccatgccgtttttcattttgagattttgcaaaacggcatgcagttcgggtaagtcggatgccgcaattaccaattttgggtcagtctgtgtaattgtcgtttcataaatccgattaacgtgtactttgaacaaaactcagcagtaaacttctttattcatc

SEQ ID NO: 2 - protein, 1118 aa, Arabidopsis thaliana
MHWIATRNAVVSFPKWRFFFRSSYRTYSSLKPSSPILLNRRYSEGISCLRDGKSLKRITTASKKVKTSSDVLTDKDLSHLVWWKERLQTCKKPSTLQLIERLMYTNLLGLDPSLRNGSLKDGNLNWEMLQFKSRFPREVLLCRVGEFYEAIGIDACILVEYAGLNPFGGLRSDSIPKAGCPIMNLRQTLDDLTRNGYSVCIVEEVQGPTPARSRKGRFISGHAHPGSPYVYGLVGVDHDLDFPDPMPVVGISRSARGYCMISIFETMKAYSLDDGLTEEALVTKLRTRRCHHLFLHASLRHNASGTCRWGEFGEGGLLWGECSSRNFEWFEGDTLSELLSRVKDVYGLDDEVSFRNVNVPSKNRPRPLHLGTATQIGALPTEGIPCLLKVLLPSTCSGLPSLYVRDLLLNPPAYDIALKIQETCKLMSTVTCSIPEFTCVSSAKLVKLLEQREANYIEFCRIKNVLDDVLHMHRHAELVEILKLLMDPTWVATGLKIDFDTFVNECHWASDTIGEMISLDENESHQNVSKCDNVPNEFFYDMESSWRGRVKGIHIEEEITQVEKSAEALSLAVAEDFHPIISRIKATTASLGGPKGEIAYAREHESVWFKGKRFTPSIWAGTAGEDQIKQLKPALDSKGKKVGEEWFTTPKVEIALVRYHEASENAKARVLELLRELSVKLQTKINVLVFASMLLVISKALFSHACEGRRRKWVFPTLVGFSLDEGAKPLDGASRMKLTGLSPYWFDVSSGTAVHNTVDMQSLFLLTGPNGGGKSSLLRSICAAALLGISGLMVPAESACIPHFDSIMLHMKSYDSPVDGKSSFQVEMSEIRSIVSQATSRSLVLIDEICRGTETAKGTCIAGSVVESLDTSGCLGIVSTHLHGIFSLPLTAKNITYKAMGAENVEGQTKPTWKLTDGVCRESLAFETAKREGVPESVIQRAEALYLSVYAKDASAEVVKPDQIITSSNNDQQIQKPVSSERSLEKDLAKAIVKICGKKMIEPEAIECLSIGARELPPPSTVGSSCVYVMRRPDKRLYIGQTDDLEGRIRAHRAKEGLQGSSFLYLMVQGKSMACQLETLLINQLHEQGYSLANLADGKHRNFGTSSSLSTSDVVSIL

SEQ ID NO: 3 - DNA, 3765 bp, Glycine max
gtcagatacagagtccttccctcctcgtgtgtggactgtggcgggaactcattttgctagtttgcttcctctctctctctcgttcccattcaacgcaatgtacagggtagccacaagaaacgtcgccgttttcttccctcgttgctgttccctcgcgcactacactccttctctatttcccattttcacttcattcgctccctctcgtttccttagaataaatggatgtgtaaagaatgtgtcgagttatacggataagaaggtttcaagggggagtagtagggccaccaagaagcccaaaataccaaataacgttttagatgataaagaccttcctcacatactgtggtggaaggagaggttgcaaatgtgcagaaagttttcaactgtccagttaattgaaagacttgaattttctaatttgcttggcctgaattccaacttgaaaaatggaagtctgaaggaaggaacactcaactgggaaatgttgcaattcaagtcaaaatttccacgtcaagtattgctttgcagagttggggaattctatgaagcttggggaatagatgcttgtattcttgttgaatatgtgggtttaaatcccattggtggtctgcgatcagatagtatcccaagagctagttgtcctgtcgtgaatcttcggcagactttagatgatctgacaacaaatggttattcagtgtgcattgtggaggaggctcagggcccaagtcaagctcgatccaggaaacgtcgctttatatctgggcatgctcatcctggaaatccctatgtatatggacttgctacagttgatcatgatcttaactttccagaaccaatgcctgtagtaggaatatctcattctgcgaggggttattgcattaatatggtactagagaccatgaagacatattcttctgaagattgcttgacagaagaagcagttgttacgaagcttcgtacttgccaatatcattacttatttttgcatacatccttgaggcggaattcttgtggaacctgcaactggggagaatttggtgagggagggctattatggggagaatgtagttctagacattttgattggtttgatggcaaccctgtctccgatcttttggccaaggtaaaggaactttatagtattgatgatgaggttacctttcggaacacaactgtgtcttcaggacatagggctcgaccattaactcttggaacatctactcaaattggtgccattccaacagaaggaataccttctttgttgaaggttttacttccatcaaattgcaatggattaccagtattgtacataagggaacttcttttgaatcctccttcatatgagattgcatccaaaattcaagcaacatgcaaacttatgagcagtgtaacgtgttcaattccagaatttacatgtgtttcgtcagcaaagcttgtaaagctacttgaatggagggaggtcaatcatatggaattttgtagaataaagaatgtactggatgaaattttgcagatgtatagtacctctgagctcaatgaaatattgaaacatttaatcgagcccacatgggtggcaactgggttagaaattgactttgaaaccttggttgcaggatgtgagatcgcatctagtaagattggtgaaatagtatctctggatgatgagaatgatcagaaaatcaactcgttctcttttattcctcacgaattttttgaggatatggagtctaaatggaaaggtcgaataaaaagaatccacatagatgatgtattcactgcagtggaaaaagcagctgaggccttacatatagcagtcactgaagattttgttcctgttgtttctagaataaaggctattgtagcccctctcggaggtcctaagggagaaatatcttatgctcgggagcaagaagcagtttggttcaaaggcaaacgctttacaccgaatttgtgggctggtagccctggagaggaacaaattaaacagcttaggcatgctttagattctaaaggtagaaaggtaggggaggaatggtttaccacaccaaaggtcgaggctgcattaacaaggtaccatgaagcaaatgccaaggcaaaagaaagagttttggaaattttaaggggactcgctgctgagttgcaatacagtataaacattcttgtcttttcttccatgttgcttgttattgccaaagctttatttgctcatgcaagtgaagggagaagaaggagatgggtctttcccacgcttgtagaatcccatgggtttgaggatgtgaagtcattggacaaaacccatgggatgaagataagtggtttattgccatattggttccacatagcagaaggtgttgtgcgtaatgatgttgatatgcaatcattatttctgttgacaggaccgaatggtggtgggaaatcaagttttcttaggtcaatttgtgctgctgcactacttgggatatgtggactcatggttcctgcagaatcagccctaattccttattttgactccatcacgcttcatatgaagtcatatgatagtccagctgataaaaagagttcctttcaggttgaaatgtcagaacttcgatccatcattggcggaacaaccaacaggagccttgtacttgttgatgaaatatgccgaggaacagaaactgcaaaagggacttgcattgctggtagcatcattgaaacccttgatggaattgggtgtctgggtattgtatccactcacttgcatggaatatttactttgcccctaaacaaaaaaaacactgtgcacaaagcaatgggcacaacatccattgatggacaaataatgcctacatggaagttgacagatggagtttgtaaagaaagtcttgcttttgaaacggctaagagggaaggaattcctgagcatattgttagaagagctgaatatctttatcagttggtttatgctaaggaaatgctttttgcagaaaatttcccaaatgaagaaaagttttctacctgcatcaatgttaataatttgaatggaacacatcttcattcaaaaaggttcctatcaggagctaatcaaatggaagttttacgcgaggaagttgagagagctgtcactgtgatttgccaggatcatataaaggacctaaaatgcaaaaagattgcattggagcttactgagataaaatgtctcataattggtacaagggagctaccacctccatcggttgtaggttcttcaagcgtctatgtgatgttcagaccagataagaaactctatgtaggagagactgatgatctcgagggacgggtccgaagacatcgattaaaggaaggaatgcatgatgcatcattcctttattttcttgtcccaggtaaaagcttggcatgccaatttgaatctctgctcatcaaccaactttctggtcaaggcttccaactgagcaatatagctgatggtaaacataggaattttggcacttccaacctgtatacataactagtctatagacattgatattatctacctcaatcgcgtatttttgcctcttttaaatggctcaaagacttcaatcatcgatgttaagtttaggaaacaatgtctgcagcatttttgttagaattagttgctgcagctgcatttatgtccacatcttcaagtgtggaaattcttgttcattagcttgtaagtacaaaagtgtttgtgtacgtttggagtcccgagagaatatacaagtacaaatgaacaaatatattagtaatgaatgcactaga

SEQ ID NO: 4 - DNA, 3642 bp, Zea mays
gcgcactaccccgagaaacgtgcgacgggaacctccgcggttccccaagttcgcctccttcactactctcgcgccccggcacgcctgaaaaaccccacccctcctgccgctccgcctctcccatcacttcccacgcccctcgccgcctcccattccagcgtggacacgacgccactcgccagcacggagacgcgcgcctcgaagcactactgcactagccagccgtcgttcttccgcgccggcgccatgcaccgggtgctcgtgagctcgcttgtggccgccacgccgcgatggctgcccctcgccgactccatcctccggcgccgccggccgcgctgctcccctcttcccgtgctgatgttcgatcggagggcttggtccaagccaaggaaggtctcacgaggcatttcagtggcgtccaggaaagctaacaaacagggagaatactgtgatgaaagtatgctgtcgcatatcatgtggtggaaagagaaaatggagaggtgcagaaaaccatcatccatacaattgactcagaggcttgtgtattcaaatatattagggttggatccgaatttaagaaacggaagcttgaaagatggaaccctgaacatggagattttggtatttaaatcaaaatttcctcgtgaggttctactttgcagagtaggagatttctatgaagctatcggttttgatgcctgtattctcgtagagcatgcaggcttaaatccttttggaggtttgcgttccgacagtattcctaaagctgggtgtccagtcgtgaatttacggcagacattggatgatttgactcgatgtggttattccgtgtgcatagtcgaggaaattcaaggcccaactcaagcccgtgctcggaaaagtcgatttatttctgggcatgcccatcctggtagtccttatgtatttggtcttgctgaagtagaccatgatgtagagttccctgatccgatgcctgttgttgggatttcacattctgcaaaaggttattgcttgatatctgtgctagagacaatgaaaacttattcagctgaggagggcttaacagaggaggctattgttactaagctccgcatatgtcgttatcaccatctataccttcacaattctttgaagaataattcttcagggacatcacgctggggtgaattcggtgaaggtgggctcttgtggggagagtgcagtgggaagtcctttgagtggtttgacggttcacctattcaagaacttttatgcaaggtacgggaaatatatggccttgatgagaaaacggtttttcgcgatgtcaccgtctcattggaaggcaggccccaacctcttcatcttgggactgctactcaaattggagtcataccaactgagggaataccgagtttgttaagaatggtgcttccttcaaattgtggcgggcttccatcaatgtatattagagatcttcttcttaatcctccatcatttgaggttgcagcagcgatccaagaggcttgcaggcttatgggcaacataacctgctccattcctgaatttacatgcatatcagcagcaaagcttgtgaaactacttgagtcgaaaggggtcaatcacattgaattttgtagaataaaaaatgtccttgatgagattatgctcatgaacagggatgctgagctttctgcaatcctgcatgaattactggtacctgcttctgtggctactggtttcaaagttgaagctgatatgctaatgaacggatgtagcattatttcacaacgaatagctgaagtgatttctttaggtgttgaaagtgatcaggcaataacttcattggaatatattccaaaggagttcttcaatgatatggagtcatcttggaaggggcgcgtgaaaaggatccatgctgaagaagagtttgcaaatgttgatagggctgctgaggcattatcaattgcggtcattgaagattttatgccaattatttcgagggtgaaatctgtagtgtcctcgaatggaggtttgaaaggagaaatcggttatgcaaaagaacatgaagctgtttggtttaaaggaaagagattcataccaaatgtatgggctaacacacctggtgagcagcaaataaaacaactgaagcctgcaattgattcaaaaggcagaaaggttggggaggaatggtttacaacaagcaaagttgagaatgctttagccaggtaccatgaagcttgtgataatgcaagaaataaagttcttgagctgttgagaggcctttctagtgaattgcaggacaaaattaacatacttgtcttttgctcaacactgctcatcattgcaaaagcactttttggtcatgttagtgaggctcgaagaagaggttggatgcttcctactatatctcccttatcaaaggactgtgttgtggaggaaagttcaagtgcaatggatttagtaggactatttccttactggcttgatgttaatcaaggaaatgcaatattgaatgatgtccacatgcactctttatttgttcttactggcccaaatggtggtggtaaatctagcatgttgcgatcagtctgtgcagctgtgcttcttggaatatgtggcctgatggtaccttcaacttcagctgtaatcccacattttgattccattatgctgcatatgaaagcctatgatagcccagcagatgggaaaagttcatttcagattgaaatgtcggagatacgtgctttagtcagccgagctactgctaggagtcttgttctgattgatgaaatatgtagaggcacagaaactgcaaaaggaacatgtatagctggtagcatcattgaaagacttgataatgttggctgcctaggcatcatatcaactcacctgcatgggattttcgacctgcctctctcacttagcaacactgatttcaaagctatgggaactgaagtggtcgatggatgcattcatccaacatggaaactgattgatggcatatgtagagaaagccttgcttttcaaacagcaaggagggaaggcatgcctgacttgataatcaccagggctgaggagctatatttgagtatgagtacaaataacaagcagggagcatcagtggcgcacaatgagcctcctaatggcagccccagtgtaaatggcttggttgaggagcctgaatctctgaagaacagactagaaatgctgcctggtacctttgagccgctgcggaaggaagttgagagtgctgttactacgatgtgtaagaaaatactgtcggacctttacaacaaaagtagcatcccagaactggtcgaggtggtctgcgttgctgtaggtgctagagagcaaccaccgccttccactgttggcagatctagcatctacgtgattatcagaagcgacaacaggctctatgttggacagacggacgatcttctggggcgcttgaacgcccacagatcgaaggaaggcatgcgggacgctacggtattatacgtcttggtccctggcaagagcgttgcctgccagctggaaacccttctcataaaccagctcccttcgaggggcttcaagctcatcaacaaggcagacgggaagcacaggaacttcggtatatctcgaatctctggcgaggcagttgctactggacggaactag

SEQ ID NO: 5 - DNA, 3373 bp, Lycopersicon esculentum
atgtattgggttacggcaaaaaacgtcgtcgtttcagttccccgttggcgttcactgtcccttttcctccgtccaccacttcgccggcgtttcttatctttctctccacatactctgtgccgagagcagatacgttgcgtgaaggagcggaagttttttgccacaacggcaaaaaaactcaaacaaccaaaaagtattccagaggaaaaagactatgttaatattatgtggtggaaagagagaatggaattcttgagaaagccttcttccgctcttctggctaagaggcttacatattgtaacttgctgggtgtggatccgagtttgagaaatggaagtcttaaagagggaacacttaactcggagatgttgcagttcaagtcaaaatttccacgtgaagttttgctctgtagagtaggtgatttttatgaagctattggattcgatgcttgtattcttgtggaatatgctggtttaaatccatttggtggcctgcactcagatagtataccaaaagctggttgtccagttgtgaatctaagacagacgcttgatgatctcacacgtaatggtttctctgtgtgcgtcgtggaggaagttcagggtccaactcaagctcgtgctcgtaagagtcgatttatatcagggcatgcacatccaggcagtccctatgtttttggccttgttggagatgatcaagatcttgattttccagaaccaatgcctgttgttggaatatcccgttcagcgaaggggtattgcattatctctgtttacgagactatgaagacttactctgtggaagatggcctaactgaagaagccgtagtcaccaaacttcgtacttgtcgatgccatcatttttttttgcataattcattgaagaacaattcctcaggaacatcgcgttggggagagtttggtgaaggtggacttttgtggggagaatgtaatgctagacagcaggaatggttggatggcaatcctatcgatgagcttttgttcaaggtaaaagagctttatggtctcaatgatgacattccattcagaaatgtcactgttgtttcagaaaataggccccgtcctttacaccttggaactgccacacaaattggtgctattccaaccgaagggattccatgtttgttaaaggtgttgcttcctcctcattgcagtggtctaccagtcctgtatattagggatcttcttttaaatccaccagcctatgagatttcttcagacattcaagaggcatgcagacttatgatgagtgtcacatgttcaattcctgattttacctgtatttcatctgcaaagctggtcaagctgcttgagttgagggaggcaaatcacgttgagttctgcaaaataaagagcatggtcgaagagatactgcagttgtatagaaattcagagcttcgtgctattgtagagttactgatggatcctacttgggtggcaactgggttgaaagttgattttgatacactagtaaatgaatgtggaaagatttcttgtagaatcagtgaaataatatccgtacatggtgaaaatgatcaaaagattagttcctatcctatcatcccaaatgatttctttgaagatatggagttgttgtggaaaggccgtgtcaagaggatccatttggaggaagcatatgcagaagtagaaaaggctgcggatgctttatctttagccataacagaagatttcctacctattatttcaagaataagggccacgatggccccacttggaggaactaaaggggagattttgtatgcccgtgagcatggagctgtatggtttaagggaaagagatttgtaccaactgtttgggctggaaccgctggagaagaacaaattaagcaactcagacctgctctagattcaaaggggaagaaggttggagaagaatggttcactacaatgagggtggaagatgcaatagctaggtatcacgaggcaagtgctaaggcaaagtcaagggtcttggaattgctaaggggactttcttctgaattactatctaagatcaatatccttatctttgcatctgtcttgaatgtgatagcaaaatcattattttctcatgtgagtgaaggaagaagaagaaattggattttcccaacaatcacacaatttaacaaatgtcaggacacagaggcacttaatggaactgatggaatgaagataattggtctatctccttattggtttgatgcagcacgagggactggtgtacagaatacagtagatatgcagtccatgtttcttttaacaggtccaaatggtgggggcaaatcaagcttgctgcgttcgttgtgtgcagctgcattgctaggaatgtgtgggttcatggttccagctgaatcagctgtcattcctcattttgactcaattatgctgcatatgaaatcatatgatagtcctgttgatggaaaaagttcatttcagattgaaatgtctgaaattcggtctctgattactggtgccacttcaagaagtcttgtacttatagatgaaatatgtcgaggaacagaaacagcaaaagggacatgtattgctggaagtgtcatagaaaccctggacgaaattggctgtttgggaattgtatcaacccacttgcatggaatatttgatttacccctgaaaatcaagaagaccgtgtataaagcaatgggagctgaatatgttgacggtcaaccaataccaacttggaaactcattgatgggatctgtaaagagagtctagcatttgaaacagctcagagagaaggaattccagaaatattaatccaaagagcagaagaattgtataattcagcttacgggaatcagataccaaggaagatagaccaaataagacctctttgttcagatattgacctcaatagcacagataacagttctgaccaattaaatggtacaagacaaatagctttggattctagcacaaagttaatgcatcgaatgggaatttcaagcaagaaacttgaagatgctatctgtcttatctgtgagaagaagttaattgagctgtataaaatgaaaaatccgtcagaaatgccaatggtgaattgcgttcttattgctgccagggaacagccggctccatcaacaattggtgcttcaagtgtctatataatgctaagacctgacaaaaagttgtatgttggacagactgatgatcttgagggcagagtacgtgctcatcgcttgaaggagggaatggaaaacgcgtcattcctatatttcttagtctctggcaagagcatcgcctgccaattggaaactcttctaataaatcaacttcctaatcatggttttcagctaacaaacgttgctgatggtaagcatcgtaattttggca

SEQ ID NO: 6 - DNA, 3180 bp, Sorghum bicolor
atgcaccgggtgctcgtgagctcgctcgtggccgccacgccgcggtggctccccctcgccgactccatcctccggcgccgccgcccgcgctgctctcctcttcccatgctgctattcgaccggagggcttggtccaagccaaggaaggtctcacgaggcatctcagtggcgtctaggaaagctaacaaacagggagaatattgtgatgaaagcatgctatcgcatatcatgtggtggaaagagaaaatggagaagtgcagaaaaccatcatccgtacaattgactcagaggcttgtgtattcaaatatattagggttggatccaaatctaagaaatggaagcttgaaagatggaaccctgaacatggagattttgctatttaaatcaaaatttcctcgtgaggttctactttgcagagtaggagacttctatgaagctattggttttgatgcctgtattctcgtagagcatgcaggcttaaatccttttggaggtttgcgttctgacagtatccctaaagctgggtgtccagtcgtgaatttacggcagacattggatgatttgactcgatgtggttattctgtgtgcatagttgaggaaattcaaggcccaacacaagcccgttcccggaaaagtcgatttatttctgggcatgcccatcctggtagtccttatgtatttggtcttgctgaagtagaccatgatgtagagttccctgatccgatgcctgttgttgggatttcacattctgcaaaaggttattgcttgatatctgtgctagagacaatgaaaacttattcagctgaggagggcttaacagaagaggctattgttactaagctccgcatatgtcgttatcatcatctataccttcacaattctttgaagaataattcttcagggacatcacgctggggtgaattcggtgaaggagggctcttgtggggagagtgcagtgggaagtcctttgagtggtttgatggtttacctattgaagaacttttatgcaaggtacgggaaatatatggccttgatgagaaaactgtttttcgcaatgtcaccgtctcattggaaggcaggccccaacctctttatcttggaactgctactcaaattggagtcataccaactgagggaataccgagtttgctaaaaatggcactcccttcaagttgtggcgggcttccatcaatgtatattagagatcttcttcttaatcctccatcatttgatgttgcggcagcggtccaagaggcttgcaggcttatggggagcataacttgttctgttcctgaatttacttgcatatcacttgtgaagctacttgagtctaaagaggtcaatcacattgaattttgtagaataaaaaatgtccttgatgagattatgctcatgaacaggaatgctgagctttctgcaatcctgaacaaattgctggtacctggttctgtggctactggtttgaaagttgaagctgatatgctagtcattgaagattttatgccaattatttcaagggtgaaatctgtagtgtcctcaaatggaggttcgaaaggagaaatctgttatgcaaaagaacatgaagctgtttggtttaaaggaaagcgattcacaccaactgtatgggctaacacacctggtgagcagcaaataaaacaactgaagcctgcaattgattcgaaaggcagaaaggttggggaggaatggtttacaacaagcaaagttgagaatgctttagccaggtaccatgaagcttgtgataatgcaagaaataaagttgttgagctgttgagagggctttcaagtgaattgcaggacaaaattaacatacttgtcttttgctcaacactgctcatcattgcaaaagcactttttggtcatgttagtgaggctcggagaagaggctggatgcttcctactatatttcccttgtcaaaggactgtgttgcagaggaaagttcaaatgcaatggatttagtaggactctttccttactggcttgatgttaatcaaggaaatgcaatattgaatgatgtccacatgcactctttatttgttcttactggtccaaatggtggtggtaaatctagtatgttgcgatcagtctgtgcagctgcgctgcttggaatatgtggcctgatggtaccttcaacttcagctgtaatcccgcattttgattccattatgctgcatatgaaagcctacgatagcccagccgatgggaaaagttcatttcagattgaaatgtcggagatacgtgctttagtcagccgagctactgctaggagtcttgtcctgattgatgaaatatgtaggggcacagaaactgcaaaaggaacctgtattgctggtagcatcatcgaaaggctggataatgttggctgcctaggcatcatatcaactcacctgcatgggatttttgacttgcctctctcactcagcactactgatttcaaagctatgggaactgaagtggtcgacgggtgcattcatccaacatggaaactgatggatggcatctgtagagaaagccttgcttttcaaacagccaggagggaaggcatgcctgagttcataatcagaagggctgaggagctatatttgactatgagtacaaataacaagcagaccgcatcaatggtccacaatgagcctcgtaatgacagccccagtgtaaatggcttggttgagaagcctgaatatctgaaatacagactagaaattctgcctggtacctttgagccgttgcggagggaagttgagagtgctgttactatgatatgcaagaaaaaactgttggatctttacaataaaagtagcatcccagaactggttgaggtggtctgtgttgctgtaggtgctagagagcaaccaccaccttccactgttggcaggtctagcatctatgtgattatcagaagcgacaacaagctttatgttggacagacggatgatcttctggggcgccttcacgcccacagatcgaaggaaggcatgcaggatgctacgatattatacatcttggttcctggcaagagcgttgcctgccagctggaaacccttctcataaatcagcttccttcgaggggcttcaagctcatcaacaaggcagacggaaagcataggaacttcggtatatctcgaatctctggagaggcaatcgccacccagctaaactaa

SEQ ID NO: 7 - DNA, 3399 bp, Oryza sativa
atggccattcagcggctgctcgcgagctcgctcgtggccgccacgccgcggtggcttcccgtcgccgccgactcgtttctccggcgccgccaccgccctcgctgctccccgctccccgcgctgctatttaacaggaggtcctggtctaaaccaaggaaagtctcacgaagcatttccattgtgtctaggaagatgaacaaacaaggagatctctgtaatgaaggcatgctgccacatattctgtggtggaaagagaaaatggagaggtgcaggaaaccatcatcaatgcaattgactcagagacttgtgtattcaaatattttaggattggatccaactttaagaaatggaagcttgaaggatggaagcctgaacacggaaatgttgcaattcaaatcgaagtttcctcgtgaagttctactttgcagagtgggagatttctacgaggctgttgggtttgatgcatgtatccttgtggagcatgcaggcttaaatccttttggaggcttgcgttctgatagtattccaaaagctggatgtccagtcatgaatttgcggcagacattggatgatttgactcgatgtggttactctgtgtgcatagttgaagaaattcaaggcccaacccaagctcgtgctaggaaaggccgatttatttctggccatgcacatcctggtagtccttatgtatttggtcttgctgaagtagaccatgatgttgagttccctgatccaatgcctgtagttgggatttcacgatctgcaaaaggctattgcctgatttctgtgctagagacaatgaaaacatattcagctgaggagggcttaacagaggaagcagttgttactaagcttcgcatatgccgttatcatcatctataccttcatagttctttgaggaacaattcttcaggcacatcacgctggggagaatttggcgaaggtgggctattgtggggagagtgcagtggaaaatcttttgagtggtttgatggtaatcctattgaagaactgttatgcaaggtaagggaaatatatgggcttgaagagaagactgttttccgtaatgtcagtgtctcattggaagggaggcctcaacccttgtatcttggaacagctactcaaattggggtgataccaactgagggaatacccagtttgctaaaaattgttctccctccaaactttggtggccttccatcattgtatattagagatcttcttcttaaccctccatcttttgatgttgcatcatcagttcaagaggcttgcaggcttatgggtagcataacttgctcgattcctgaatttacatgcataccggcagcaaagcttgtgaaattactcgagtcaaaagaggttaatcacatcgaattttgtagaataaagaatgtcctcgatgaggtgttgttcatgggtagcaatgctgagctttctgctatcctgaataaattgcttgatcctgccgccatagttactgggttcaaagttgaagccgatatactagtgaatgaatgtagctttatttcacaacgtatagctgaagtaatctctttaggtggtgaaagtgaccaggcaataacttcatctgaatatattccgaaagagttcttcaatgatatggagtcatcttggaagggacgtgtaaaaagggtgcatgctgaagaggagttctcaaatgttgatatagctgctgaggcactgtcaacagcggtcattgaagattttctgccaattatttcaagagtaaaatctgtgatgtcctcaaatggaagttcgaagggagaaatcagttatgcaaaagagcatgaatctgtttggtttaaagggaggcgattcacaccaaatgtgtgggccaacactcctggtgaactacagataaagcaattgaagcctgcaattgactcaaaaggtagaaaggtcggagaagaatggttcaccactatcaaagttgagaatgctttaaccaggtaccatgaagcttgtgataatgcaaaacgtaaagttcttgagttgttgagaggactttcaagtgaattgcaggacaagattaatgtccttgtcttttgctcaacgatgctcatcataacaaaagcactttttggtcatgttagtgaaggacgaagaaggggttgggtgcttcctactatatctcccttgtgtaaggataatgttacagaggaaatctcaagtgaaatggaattgtcaggaacttttccttactggcttgatactaaccaagggaatgcaatactgaatgatgtccatatgcactctttgtttattcttactggtccaaacggtggtggtaaatccagtatgctgagatcagtctgtgctgctgcattacttggaatatgtggcctgatggtgccagctgcttcagctgtcatcccacatttcgattccatcatgctgcatatgaaagcatatgatagcccagctgatggtaaaagttcgtttcagattgaaatgtcagagatacgatctttagtctgccgagctacagctaggagtcttgttctaattgatgaaatatgtaggggcacagaaacagcaaaaggaacatgtatagctggtagcatcattgaaagactcgataatgttggctgcataggcatcatatcaactcatttgcatggcatttttgaccttccactgtcactccacaatactgatttcaaagctatgggaaccgaaatcatcgataggtgcattcagccaacatggaaattaatggatggcatctgtagagagagtcttgcttttcaaacagccaggaaagaaggtatgcctgacttgataattagaagagctgaggaactatatttggctatgagcacaaacagcaagcagacatcatcagctgtccaccatgaaatatccatagccaactctactgtaaatagcttggttgagaagcctaattacctgagaaatggactagagcttcaatctggttccttcggattactaagaaaagaaattgagagtgttgttaccacaatatgcaagaagaaactgttggatctctacaacaaaaggagcatctcagaactgattgaggtggtctgtgttgctgtgggtgctagggagcaacccccaccttcaactgttggcaggtccagcatttatgtaattatcagacgtgacagcaagctctatattggacagacggatgatcttgtgggtcgacttagtgctcacagatcgaaggaaggtatgcaggatgccacgatattatatattttggtacctgggaagagcattgcatgccaactggaaactcttctcataaatcagctacctttgaaaggtttcaagctcatcaacaaggcagatggcaagcatcgaaatttcggtatatctcttgtcccaggagaggcaattgccgcatag

SEQ ID NO: 8 - DNA, 3381 bp, Brachypodium distachyon
atgcagcggcttctggcgagcacgatcgtggccgccacgccgcgttggctccccctcgccgactctatcgtccggcgccgccgcccgcgccgttccccgctccccgtcctgctattccacagatcattgtacaaaccaaggaaggtttcacgaggcattacaatggtgtctaataaggtgaacaaacagggagatctctgcaatgaaggcatgctgtcacatattatgtggtggaaagagaaaatggagagctgcaggaaaccatcatctgtgcagttgactcagagacttgtgtactctaatatattagggttggatccaactttaaggaatggaagcttaaaagatggaaccctgaacatggagatgttacaatttaaatcaaagtttccacgtgaggtcctactttgcagagtaggagatttctatgaagccattgggtttgatgcctgcattcttgtagagcatgcaggcctaaatccttttgggggcttgcgttctgacagtattccaaaagctggatgtccaatcatgaatttgcggcaaacattggatgatttgactcggtctggttattctgtgtgcatagttgaggaaattcaaggcccaactcaagcccgtgctcggaaaggtcgatttatctctggccatgcgcatcctggcagtccttatgtatttggtcttgctgaagtagatcatgatcttgagtttcctgacccaatgcctgtagttgggatttcacgctctgcaaaaggctattgcttgatttctgtgctagagacgatgaaaacttattcagctgaggagggcctaacagaagaagctgtagtgactaagctgcgcatatgccgttatcatcatctataccttcacagttctttgaggaataattcttcagggacatcacgctggggggaattcggagagggaggactcttgtggggagagtgcagtggaaagtgttttgaatggtttgatggttctcctattgaggaacttttatgcaaggtaagggagatatatgggctggatgagaaaactaatttccgcaatgtcactgtctcattggaagggaggcctcaacctttatatcttggaactgctactcaaattggagtgatacaaacggagggaattcccagtttactaaaaatgctactccctccaaactatggcgggcttccatcaatgtatatcagagatcttcttcttaatcctccatcttttgatgtcgcgtctgcaattcaggaggcttgcaggcttatgggcagcataacttgttcgattcctgaatttacttgcataccatcagcgaagcttgtgaaattactcgagtcaaaagaggttaatcacattgaattttgtagaataaagaatgtccttgatgacattatattaatgaatggaaacactgagctttctgctatcatggacaaattgctcgaacctgcttcggtggttactggtttgaaagttgatgctgatatactaattagagaatgtagccttatctcacaacgtataggtgaagtcatctctttaggtggggaaagcgatcaggcaataacttcatcggaatatattcccaaggagttctttaatgatatggagtcatcttggaaggggcgtgtgaaaagggttcatgctgaagaagagttcacaaatgtcgatgtagctgctgaagcattatcaaccgcggtaactgaagattttctgccaattattgtaagagttaaatctgtgatatcttcacatggaggttctaaaggggaaatctcttatgcaaaagaacacgaagctgtttggtttaaagggaagcgattcacaccaaatgtctgggcgaacacacctggtgaacaacagataaaacaactaaagcctgcgattgattcaaaaggtagaaaagttggggaggaatggtttacaacaatcaaagttgagaatgctttagccaggtatcatgaagcttgtgatagtgcaaaaggcaaagttcttgagctgttgagaggtctttcaagtgaattgcaggacaagattaatatacttgtcttctgctcgacgctgctcatcatagcaaaagcactttttggtcatgttagcgagggtcttagaaggggttgggtgcttcctgccatatctcccctatctaaggactatagtactgaagaaggctcaagtgaaatggatttattgagactctttccttactggcttgacagtaatcaagggaatgcaatactgaatgatgtcaatatgcactctttgtttattctgactggcccaaatggtggaggtaaatccagtatgttgcgatcagtctgtgcagctgcattgcttggaatatgtggtctgatggtgccagctgcttcagctgtcatcccacactttgattccatcatgctgcatatgaaggcctatgatagcccagctgatgggaaaagttcgtttcagattgaaatgtcagagatccgatctttagtcagccgtgctactggtaggagtcttgttctcattgatgaaatatgtaggggcacagaaactgcaaaaggaacttgtatagctggtagcatcatcgaaaggctcgacgatgttggctgcctaggcatcatatcaacccatttgcatggcatttttgacttgcctctgtcactcggcaatactgatttcaaagctatgggaacagaagttgtcaatgggtgcattcagccaacatggagattaatggatggtatctgtagagaaagccttgcttttcaaacagcaaggaaggaaggtatgcctgacttgataattaaaagagcagaggagctatacagtactatgggcagaagcaagacgtcatcaacagtccaccatggtccatccgttgctaagtctaaagcaagtggattggttgatatgcctgatggtctgggaaatggattagaacttccatctggtgcttttgcactgctgcgaaaggatgtcgaaataattgtgaccgcaatatgcaaggataaattgttggatctctacaacaaaagaagcatctcagagctggttgaggtggtttgtgttactgtaggtgctagggagcaaccgccaccttcaactgttggcaggtccagcatctacatagttatcaggcgtgacaacaagctctatgttggacagacggatgatcttgttggccgtcttgctgttcatagatccaaggaaggtatgcagggtgccacaatattatatatcgtggttcctggcaagagcgttgcgtgccagctggagacacttctcataaaccagcttccctcgaaaggttttaagctcacgaacaaggcagatggcaagcatcggaacttcggcatgtctgttatctctggagaagccattgctgcacactga

SEQ ID NO: 9 - DNA, 3520 bp, Vitis vinifera
atgtactggctgtcaaccaaaaacgtcgtcgtttcattccctcgattctactctctcgctcttcttctccgttcccctgcctgcaaatacacttcatttcgttcttctacacttctactccaacagtttgagaagagccgatgtctcaacgaaaggagggttttgaaaggagctggaagaatgacaaaaaatgttataggattgcaaaatgagctagatgaaaaggatctttctcacataatgtggtggaaggagaggatgcaaatgtgtaaaaagccgtccactgtccaccttgttaaaaggcttatatattccaatttgctaggagtggatcctaacttgaaaaatgggaatctaaaagaaggaacgctgaactgggagatgttgcagttcaagtcaaagtttcctcgtgaagttttactctgcagagtaggggatttttatgaagccatcggaattgatgcttgtattcttgttgaatatgctggtttgaatccttttggtggtttgcgctcagacagtataccaagagctggctgcccagtcatgaatctacgacaaactttggatgacctgacacgtagcgggtattcagtttgcatagtggaggaagttcagggtccaactcaagctcgttctcgtaaaggtcgttttatctctgggcatgcgcatccgggtagtccttatgtatttggacttgttggggttgatcatgatcttgattttccagaaccaatgcctgtagttggaatttctcgttctgcgaagggttattctataattttagtccttgagactatgaagacgttttcagtagaggatggtctgacagaagaggctttagttaccaagcttcgcacttgtcactaccatcatttattgctgcatacatctctgagacgcaactcctcaggtacttgtcgttggggagaatttggtgagggaggactattatggggagaatgtagtgctagacactttgaatggtttgaaggggatcctgtatctcaacttttgtttaaggtgaaggagctctatggttttgatgatcaagttacatttagaaatgtcactgtgtcttcagagaaaagaccccgttctttacaccttggcacagctacacaaattggtgccataccaacagagggcataccgtgtttgttaaaggtgttgcttccatcaaattgcactggtctacctcttttgtatgttagagatcttcttctcaaccctcctgcttatgagattgcatccataattcaagcaacatgcagactcatgaacaatgtaacgtgctcgattcctgagtttacttgtgtttcccctgcaaagcttgtgaagctacttgagcttagggaggctaatcatattgagttctgcagaataaaaagtgtacttgatgaaatattgcagatgcatagaaactctgatcttaacaaaatccttaaattattgatggatcctacctgggtggcaactggattgaagattgactttgacacattggtgaacgaatgtgaatggatttcagctagaattggtaaaatgatctttcttgatggtgaaaatgatcaaaagataagttaccatcctatcattccaaatgacttttttgaggacatggaatctccttggaagggtcgtgtgaagaggatccatgtagaagaagcatttgctgaagtggaaagagcagctgaggcattatctttagctatctccgaagattttctacctattatttcaagaataaaagctaccacagccccacttggaggtccaaaaggagaagttgtatatgctcgagagcatgaagctgtttggttcaagggaaaacgttttgcaccagttgcatgggcaggtactccaggggaagaacaaattaagcagcttagacctgctatagattcaaaaggtagaaaggttggattggaatggtttaccacagtgaaggtggaggatgcactaacaaggtaccatgaggctggggacaaggcaaaagcaagggtcttggaattgttgaggggactttctgcggagttacaaactaaaattaacatccttatctttgcttccatgttgcttgtcattgcaaaggcattatttgctcatgtgagtgaagggagaagaaggaaatgggttttcccctctcttgtagagttgcataggtctaaggacatggaacctctggatggagctaattggatgaagataactggtttatcaccatattggttggacgtggcacaaggcagtgctgtgcataatacagttgatatgaaatcattgtttcttttgacaggacctaatgggggtggtaaatcaagtttgcttcgatcaatttgtgcagccgcattacttggaatatgtggatttatggtgcctgcagaatcggccttgattcctcattttgattctattatgcttcacatgaaatcttatgatagcccagctgatggaaaaagttcatttcagattgaaatgtcagagatgcgatccataatcactggagccacttcaagaagcctggtgctgatagatgaaatctgccgaggaacagaaacagcaaaggggacatgtattgctggtagcatagttgaaactcttgataagattggttgtctgggtattgtatccactcacttgcatggtatatttaccttgggactgaatactaagaatgctatttgtaaagcaatgggaactgaatatgttgatggcaaaacaaaaccgacctggaagttgatagatggaatctgtagagaaagccttgcctttgaaacagctcagaaggagggaattcctgaaacaattatccgaagagcagaagagctgtatctttcaatccattcaaaagacttaattacagggggaactatttgtcctaaaattgagtcaacaaatgaaatggaagtcttacataagaaagttgagagtgcagtcaccattgtttgccaaaagaagctgaaggagctctataagcagaaaaacacgtcaaaacttccagagataaactgtgtggccattttgccaggggaacagccgccgccatcaacaattggtgcttcaagtgtgtatgtgttgtttagcactgataagaaactttatgttggagagacagatgatcttgaaggcagagtccgtgcgcatcgatcaaaggaaggaatgcagaaggcctcattcctttattttgtggtcccagggaagagcttggcatgccaactcgaaacgcttctcatcaaccagctccctgtccaggggttccaactggtcaatagagctgatggtaaacatcgaaattttggcacattggatcactccgtggaagttgtgaccttgcatcaatgagcctgcgctccttgccacccattttgtagaatggttccatctttgaaatatgtacttgaatgacaaaaaccagatgaaagtggctgcagcaattttggttttttgatgtacgttgctccacttgcattagtattatctacctgatgaaatatgcattgatattgcttgctctaca

SEQ ID NO: 10 - DNA, 3615 bp, Cucumis sativus
atggaaatatccatctatgtcgatgtggcattgtggcgggaagtatcggaaaccaagggttttctgttccggcgacgacgagttacaaacaccctcctcatttcaaaccaaaacgctttaaaacttccaatcacaacaagattgaagctcacaaaccatccatttttatccaccgccatgtactgggcggcaacacgaaccgttgtttctgcttcccggtggcgttttctggctcttttgattcgcttccctccgcgtaacttcacctcagttactcattcgccggcatttatagaaaggcaacagcttgaaaagttgcactgttggaaaagcagaaaaggttcaagaggaagcatcaaagctgctaagaagtttaaggataataatattctccaagacaataagtttctttctcacattttatggtggaaagagacggtggaatcatgcaagaagccgtcatctgtccagctggttaagaggcttgacttttccaacttgctaggtttagatacaaacctgaaaaatgggagtcttaaagaaggaactcttaactgtgagattctacagttcaaggcaaagtttcctcgagaagttttgctctgtagagttggagatttttatgaagcaattggaatagatgcttgcatacttgtggaatatgctggtttaaatccttttggaggtcagcgtatggatagtattccaaaagctggttgccccgttgtgaatcttcgtcaaactttggatgatctgacacgcaatgggttctcagtgtgcatagtggaagaagttcagggcccaattcaagctcgttctcgcaaaggacgttttatatctgggcatgcacacccaggcagtccctatgtttttgggcttgtcggggttgatcacgatcttgactttccagaaccgatgcctgtgattggaatatctcgatccgcaaggggctattgcatgagccttgtcatagagaccatgaagacatattcatcagaggatggtttgacagaagaggccttagttactaaactgcgcacttgtcaataccatcatttatttcttcacacgtcattaaggaacaactcctcaggcacttgccgctggggtgaatttggtgagggtggccggctatggggggaatgtaatcccagacattttgagtggttcgatggaaagcctcttgataatcttatttctaaggttaaagagctttatggtcttgatgatgaagttacatttagaaatgttacaatatcgtcagaaaataggccacatccgttaactctaggaactgcaacacagattggtgccataccaacagagggaataccttgtttgctgaaggttttgcttccatccaattgtgctggccttcctgcattgtatatgagggatcttcttctcaatcctcctgcttatgagactgcatcgactattcaagctatatgcaggcttatgagcaatgtcacatgtgcaattccagacttcacttgctttcccccagccaagcttgtgaagttattggaaacgagggaggcgaatcatattgaattctgtagaatgaagaatgtacttgacgaaatattacaaatgcacaaaaattgcaagctaaacaatatcctgaaattgctgatggatcctgcatctgtggcaactgggttgaaaattgactatgatacatttgtcaacgaatgtgaatgggcttccagtagagttgatgaaatgatttttcttggtagtgaaagtgaaagtgatcagaaaatcagttcttatcctattattcctaatggttttttcgaggacatggaattttcttggaaaggtcgtgtgaagaggattcacattgaagaatcttgtacagaagttgaacgggcagctgaagcactctcccttgcagttactgaagattttgtcccaatcatttctagaatcagggctactaatgcaccactaggaggtccaaagggagaaatattatatgctcgggaccatcaatctgtctggttcaaaggaaaacggtttgcaccatctgtatgggctggaagccctggagaagcagaaattaaacaactgaaacctgctcttgattcaaagggaaaaaaagttggggaggagtggtttaccacgaagaaggtggaggattctttaacaaggtaccaagaggccaataccaaagcaaaagcaaaagtagtagatctgctgagggaactttcttctgaattgttagctaaaattaacgtcctaatatttgcttccatgctactcataattgccaaggcgttatttgctcatgtgagtgaagggaggaggaggaaatgggtttttcccacccttgctgcacccagtgataggtccaaggggaaagttgcgatgaagctggttggtctatctccctattggtttgatgttgtcgaaggcaatgctgtgcagaatactattgagatggaatcattatttcttttgactggtccaaatgggggtggaaaatctagtttgcttcgatcgatttgtgctgctactttgcttgggatatgtggatttatggtaccggcagagtccgccctgattccccacttcgactcaattatgcttcatatgaaatcttttgatagtcctgctgatggaaaaagttcttttcaggtggaaatgtcagagatgagatccattgtcaatagagtaacggagagaagtcttgtacttatcgatgaaatctgtcgtggaacagaaacagcaaaaggaacttgtattgccgggagcattattgaagctcttgataaagcaggttgtcttggcattgtctccactcacttgcatggaatatttgatttgcctttagatacccaaaacattgtgtacaaagcaatgggaactgtttctgcggaaggacgcacggttcccacttggaagttgattagtggaatatgtcgagagagccttgcctttgaaacagcaaagaatgaaggaatctctgaagctataattcaaagggctgaagatttgtatctctcaaattatgctaaagaagggatttcaggaaaagagacgacagatctgaacttttttgtttcttctcatccaagccttaatggtaatggcactggaaaatccaatctcaagtcaaacggtgtgattgtaaaggctgatcagccaaaaacagagacaactagcaaaacaggtgtcttgtggaagaaacttgagagggctatcacaaagatatgccaaaagaagttgatagagtttcatagagataaaaacacattgacacctgctgaaattcaatgtgttctaattgatgcaagagagaagccacctccatcaacaataggtgcttcgagcgtatatgtgattcttagaccggatggcaaattctatgttggacagactgatgatctggatggtagggtccaatcacatcgtttaaaggaaggaatgcgggatgctgcattcctttatcttatggtgcctgggaagagcttagcttgccaacttgaaactcttctcatcaatcgacttcctgatcacgggttccagctaactaacgttgctgatggaaagcatcggaattttggcacagccaatctcttatccgacaatgtgactgtttgctcatga

SEQ ID NO: 11 - DNA, 660 bp, Gossypium hirsutum
ggcacgaggttgctattgctgcaagggaacagccacctccatcaactatcggtgcttcttgcgtatatgtcatgttcagacctgataagaaactatacattggagagacggatgatcttgatggtcgaattcgttcgcatcgttcaaaggacgggatggaaaatgcttctttcctatatttcacagttccagggaagagtattgctcgccaactcgaaactcttctaatcaaccaactcttaagtcaaggcttcccgatcgccaacttggctgacggtaagcatcagaattttggcacatccagtctctcatttgacggcataaccgtagcctaacgagttaaaatgtatatcaatacgtaatttatatcgaaattgacatagaagtggcggcagcaattttgcctttgatctcggttgctccacttgctttgtacatgcatcacccttttaaccaagggtaaagttttctagtcataatttaatagcatgtatctattaagtccattttgaggtttatatgaatcaggttttcatcattaattggttaaattctgttattagctcctctactttactaaagttgtagatttagttcttatactttaattagattatttttactctatacttttcgaatgataaaattttagtcttcatt

SEQ ID NO: 12 - DNA, 2225 bp, Oryza sativa
agaaaagctaaaatggatgaaaaaaacagagaaaaagaaatcctaccctccatagcgagcagtggtggtctgcactctgcaggcaggcaggcacccaggcctgcagctcgatggcgccgccgccgccgtcgccgccgcgatctctcacctccgtctccctccggactcctctgagccctctcctcttcctacggccagcttcttgcaatccatcggcggtctccggctcctgcagcagcggagcatgccgcggcgtgcgctgctcggcggcgaacaagccttctccttccaccgctccgggcaccgaggtaaggtagccggctagccgccccccatattcttgtttctgtgttgatcggagctcgatggctggggtgctctgggctcgtcgtcgtcggtcgatcgtcatggcttgcttcgtttcttgcagctcgacctccatggcaaagataaggagtgaggtgctgtccccgttccgctccgtgcggatgttcttctacctcgcgttcatggccagcgccgggctcggggccctcatcgcgctcacgcagctcatcccggcgctgtccagcccggcgagggcggccgccgcgggggagacgctcaagggcctgggcatcgacgtcgcggcggtctccgtcttcgcgttcctctactggcgcgagagcaaggccaaggacgcgcaggtggcgaagctcacgcgggaggagaacctgtccaggctcaggatccgcgccggcgagggccgcccgcccgtcccgctcggcgagctgaggggcaccgcgcggctcgtcatcgtcgccggccccgcggcgttcgtcaccgagtcgttccgccggagcaagccgttcttgaaggacctcatggagcgcggcgtgcttgtcgtgcccttctcgacggacggcaacgcgccggacctgcagttcgacgaggccgacgaggaggaggaggaggcggcggcggcggctgggaagatgaagcggaggctctggcagctcactccggtttacacttctgaatgggccaagtacgcgcaaagccgggatcccatgaatttagctgcttaaatttcttcttcatgtcaatcgaaattcaaatgcaaattagtatctcattttcaaatcgattgctgcttcttgcagatggctagatgagcagaagaagctagccaacgtgtcacctgattcccccgtgtgagtatcaaaaactactctgaatttgtctgaaaatataactgaagtttctgcagctgctgaactgaaaccgcatcactcttgcaggtatctctcgctccggctggacggccgcgtccgtggcagcggcgtcgggtacccgccgtggcaagcgttcgtggcgcagctgccgccggtgaaggggatgtggtccggcctccttgatgggatggacgggagggtgctttgaatatttgactgatacagaccgtgaaaacattagttgattggagaaaaaaaaggacggccgggttcgatctatagcttatactagaacaagaacaggaagagtttgatgattgctttaacttctgtggggttgattttgcttcctgcatcccagcgacatcgcccaagtgaatgtgatatgccatgtgcccatgtacatgttgttttgcagcctacgtgacttgattattaacgagaatcctgtgtcaaagatcgctttttccgtggtaggcttctccattttattttatttttgaatatatatacgaaccgtgacaaatctgatggaacactggaccatgggggtaatgatactgtagtcgcctggtctttttatcaggcgctaaatgcaaacaatcagacagcttaaacaacctgaggttgttcagccagcccagaatacaaaaagcccatggaccgtgagcccgtgaaaccatggcccacccatcagtcacgtcacgtcgggacgtgtgcgcactaccccgagaagcgcgcggccgtaagccacaaccacaaccccacaccgcctcttggctgctcgcgccctgacacttcccaaaaccccaaaccgcccatatctctctcctcttctccgctcctcgcttcccccaaaaccctcgcggtggcggtgggccgccggtctcattccgccggcgtccacggaggcggccggagccaggcgctccgcgggccggggagccaccggaaggctggaaccctagcggcggcgggtctcctccccctccccgcgcgccgggcggcgcc

SEQ ID NO: 13 - DNA, 2000 bp, Solanum lycopersicum
cacgcatcaacatgtactagctaactttgtccaccaaggaatatctattaccttcaaccagcaacaagtatcagctaactttgtccatttaggttaaaaccttgactaaatccattgaaaacctattacctcccaccagcaacttatgccaactaacattgtctaccaagggatatccgttgcctcaacattgtccatcgagggatatccattgcctcccagcagcaacaagtaccagctaacattgtccaatcgagggacatccataccaaataatttttgagaaagtaattatttagggtgatgtttatttgtgcttggaaaacaaatagccattgaattagtaaaatttgcaattaaatcacattacaaaaatgtctaaggtaatttatcctaaatacaatagtgatatcaataataatatatttgagtgtaatgtcataatcaagaatttataaaaataatatgtcagtaggtttaattactgatatattaaaattgtttcgataaattcttgatttaaagagtacaatcaacaaataaaagaacaaatagtaaaatataagatacgtatatttttaaatagtagtgtacagtaggactagatgacaaaataaaattgtaagaagaagaggatagtctttaccattctcacacaaaatcatatctcgtcacaaatgaatttacagttactcataaatatatttaataaaatgatagtattagcaaaacataattgatgtgttagttcatcagttattatgcacttaaagttatttataaaaaaaaaaggtcaaatgccccccctaatctgttgtccgatttctaagtacgtacgtaaactttagaggggtcatatcacccctgaactgtttaaaattgaaatttttgtactcctaaaaagccataaccatatttatgttgatgagtgaaactcacgcgttttgacacatgaaaaatccattagaaaaagtttttcttcaattttttcattattctttattcttttcttctattttttcaccatctctccaacacaaaaatattttcactattttctccattatcataaacaccaaaggttcactaatcactacaatcttcaaaacgaaaaggtcggcagtgattttgattcttatttgtcatttcgcccactacttagttggtgctaagatcattttcatgaatacatgtgtcaaatttctcaaattagagtaaatgaataacaatggaggaaagtcgaatgtgggttttattaaaaatttaaaattcttcgtttgtttgaattaaaattacaaatttggagctttgaagaaccaaaaaaagaatttgccgacctaattgaccttaatttgtcgtttgaccatgtacaaggatgattaacaactccaataatatcgataaagagttgattttcaaaaactcttaattccatacacaaattaaaatcaagaaaaatgcgaaaattttatgaacaaatctaataacaaagaacgaaaaaatttctacgaagaacaaagaaaagaataaggaagaagataaaatatttgttttggtgctcactctatcagggagtgaaatacattcactatggagatgataatttcaattttaaacagttcaggaaggtgatatgcgtaaagtttaagttaatagataatcaaagatatctgttgacgtattgattcaatgttaaatatacagttgagttacttataacttataaatacaataagtaatttttttccttctaccatttgaaaaaaaataacgcgtacgtcattgtcttcaatcatcaacgatttattattttcaatgtgattatattattaagtaattaattcgtcccaaataccaatatctactaacattctttgcctaatgtttaattgtaattcctacagattttatttttttgaaaataatataaagtacaccatttctctgccgggaagaacaaatacacagagagagagtgtattgtgcactgatatcgagca

SEQ ID NO: 14 - DNA, 2000 bp, Sorghum bicolor
tggcacataagtaaaattgctgacttggtagggtcatttaatgaaggaatttcatgagatgagagagaagtttcatccccatgaaactcatatggctcggttacttggtaactgtgtcatcaaactatgcattgagactggcctgcatgtttcatgagagtgtcatgcacattaaataagatatcacataagcaaaattgctgacttagctgggtcattaaatgaaggagtttcatcagatgagagaggagtttcatcttcataaaactcttgtggctcggttacctagtttttagtctcggtaactgtgtcatgaaactataatacatgttttatggaagtgtcacgcatattatagggtgccacataagtaaaattgttaacttgacagagtcattaaatgaagaagtttcatcagatgagagaggagtttcatccccataaaattcatgtggctcagttacctagtttatagtcttggtaactgtgccatgaaactatgcattgagactagcctaacaaggtgataaggccagtctcaatgcatgtttcataagagtgtcatgcacattaaataagatgccacataagcaaaattgctgacttgacagggtcattaaatgaaggagtttcgttagatgagagaggagtttcatccccatgaaactcttatggctcgattacctagtttatagtcttgataactgtgtcatgaaactatgtattaagactggagactcaaatacaaattgtatatagcctatggctctatttgtttccgcgaccggccaacccgtgaccacgattaagcaaacacgactcgagatcgtgtatgtataaatttggatcttcggtggtttaattttagtttttttagctaagagaatttatatacattttccattattaaaccatgtttcaaggtttctaattccatgctctaaaataatatattattttatggaaaatagatatttttgaaattaaatgtatgtataaattttcaagactatataaaataataaaagctctaatctattgatgtagttcaatttttatctccctagagctgatgtggcaccacatacggtgccacctaggttaaaactaacctcaaaacccggctaggtttgtgatttgcctcgtatttgatagtttagggtgtactccgtataagattatctgtatattcagagattagaaaatcaaacacatctactaaattttagaacaagcatcaccctgtttggcggctagtcgtaaaagtaactgatgttaatttattgtgagagtaaaatactgttgtttgataataaaacttttacttataatttcaagctaatagagcccataaagacaaacctgtctcacaagttagaattcttacaacttttcgtctaatcacatcgaatatttgaacacatgtatatagtattaaatataataaaaatatttaattgtacagtttacctatatttacaagacgaatattttaaatataattagtttattattaaacactaattactataattataaatatactacaatataaaaaaaaaactttcgtttttgcgagctaaacaccgggacacaaaacgctcctgtctcctgggcggcttgggcctgccagagcccgggaaccgtgagcccgtgaccccagcgggcccaaccagtcagacgagagtcgaaaggcgtgcgcactaccccgagaaacgtgcgacaggaacctcccccttcccggcctgggagcggcctggcgagtggcgactggcgtcttccgcggttccccccagttcgcctccttcactgccgcccgcgcgccccgacacgcctgaaaaaccccacctctcccctccgctccgcctctctcgccctccacttcccacgccccacgccgcctgccattccagttccagcgtggactcgacgccagcgcggagacgcgcgtctcgaagcactagccccccgttgttctgccgcgccggcgcgccggcgcc

SEQ ID NO: 15 - DNA, 2049 bp, Arabidopsis thaliana
catatgaaacatttcctgtagcagtgagatggttacaagaggatccatacccgagtgctgtgcaatcagacaaactacaagcatagtcgatattatcaggcaagtcatcgaggttatatgcattagggtcaagaatacaccaagttttgggcagatacttcacatcttccacaggaaccaaaggcttgtcatttcctttacctgacaagtcaagctcatatttcggtctcccatcaaactcaaagatcccccagtgcctctcaaaagtccccggtgctatactcttggcgtcctcatcaacaaggctgaaaaggtaaacatccataatcactcctttcctcgcaggcgttccatttccagacatagcatgctttaccattccctgattgaatctctttgcactctttacattagcgttcttgtctccatccgtaggccacccgacctctcctacaatgatcttcatccccaagaagctatatctctccatagcacaaatcaaagtgtcgagattcgcatcaaacacattggtgtagaccaaatttccatctctcaaagacttgttagtcccatcaaagaaggcaaaatccaaaggaaagtaagcatttccatagagactaagaaaagggtatatgttaaccgtgaaaggcgaatcatgtgaatacaagaaattgattatctcaatcgttgcatcccttagctcaggtctaaagtctccagctgatggaacagggttcgcttcaggggaaaaatagatgtctgcgttgaaaggaacagtgactttcacatttttcagatcagcttcctctagtgctcgttggatgttgataagagctggtaatgtgaactcaacgtaagttccattatatgtctgaaggaaaggctcgtttccaacagctatgtacttgatgttgactccaccgttgtaagaataagcagtaacgttttcttcaacccatgaagctgctacagatgtatcttgagccatttctttaagaaaccggtttggtattcctatcatgacttcaatgtctgagccaattagagcgtctaagatgttttggtcggcttcaaatagtttcagcttagtgaaactattgtccattagcatcttcacaaccttttctggtggaagctggtgactcgccattattccccagttaactcctacattactcgtgttgcttgaggcaatggaaacttgtgagatgataagaaagtaacaaagaataatctgatgattataaaagtggtttgttgttaactttgatctctctcctgccatttttttctctgtttatgagtcttttcttctcttttctttatggagtctttgttaagggagaagatgaaatgtgattggatatttgtgatttgtacttagttcagttaaagaagcagacacaacatgcaaaatagccattggtgaaacactttgtgcatgcctatctgataaatccattgactcaccacaaattcttatgtaattctagatgtttcgtatttgttgtgccaaacaaacacacacactcacacactgcactgagtctagacatttagtggttttgttttcttattattaatactcattagagtattaagtttgtatagaattcagaaacaactgatagtcattttaagatttctaattacaaaacttttgatcctctttgaaaagcagagaaattacaatctttacaaacaaaactgagagattagagatgtgttcatagagatgggttctttgttagacattccaaaaagatacaaaactagccgatgattaattttggtaaattaatgaacaagaatgtaatttgaaacattatagggagcaaatgagaaattactctttttaaaaggctaaaatcctaattacctttaaactaagaagacaagaagagaagagaaaacatgttttccattagaggactgtgagattgtgaattgcatagtcgtcgtcttctggcgggaaaagaagccctagaaaaagggtgaaaggtgaaaactctacttcttcttcttcttcttcttcagagtgtgagagag

SEQ ID NO: 16 - DNA, 946 bp, Arabidopsis thaliana
aaaagttgaaacagcaaagtagcgatagatttcgtgaaaacagagaagcggacatatcttgaaacacatggcagcgatttctccatggttatcttctcctcagagcttttcgaatccccgcgttaccattacagattccagaagatgttcatcaatttctgcggcaatctctgttcttgacagctccaacgaggaacaacatcgaatttcgtctagagatcatgttgggatgaagagaagagacgtcatgttacagatagcttcctctgttttcttccttccattggccatttcacctgcatttgcagagacaaatgcatcagaagctttccgtgtgtacacagatgaaacgaacaaattcgagatatcaatcccacaagattggcaagtcgggcaagcagaacctaatggattcaagtcaatcacagctttttacccacaagaaacttcaacttccaatgtgagtatagcgatcactggactaggtccagacttcaccaggatggaatcattcggaaaggtcgaagctttcgccgaaacattggtcagtggattggatagaagctggcaaaaaccagtaggagtgactgcaaagctaatcgatagcagagcttctaagggattctattacatcgagtacaccttacaaaaccctggagaagctcgcaagcatttgtactctgcaattggaatggcaacaaacggatggtacaaccgtttatacactgtcacaggacagtttacagatgaagaatctgctgaacaaagctctaagatccagaagacagtcaagtctttcagattcatctgagaatgtcattcatatctatcagcggaactaaattatagaattgatcaaacaatttgtttactgaacaattacttttttgcaatgaaattctgagaaaagagcctactccatactttgaagtaagcttcagtaaac

SEQ ID NO: 17 - DNA, 807 bp, Arabidopsis lyrata
tccagaagatgttcatcaattcctgtagcaatctcagctctagacagctccaacgaggaacaacatcgaatttcgtctagagatcatgtggggattaaaagaagagaagccatgttacagatagcttcctctgttttcttccttccattggccgtttcacctgcatttgcagagacaaatgcatcagaagctttccgtgtgtacacagatgaagcgaacaaattcgagatatcaatcccacaagaagattggcaagtcgggcaagcagaacctaatggattcaagtcaatcacagccttttaccctcaggaaacttcaacttccaacgtgagcatagcgatcactggactaggtccggacttcaccaggatggaatcttttggaaaggtcgaagctttcgctgaaacactggtcagtggattggatagaagttggcaaaaaccagcaggagtgactgcaaagctaatcgatagcagatcttccaagggattctattacatcgagtacaccttacaaaaccctggagaagctcgcaagcatctgtactctgcaattggaatggcaacaaacggttggtacaaccgcttatacactgtcacaggacagtttacagatgaagaatctgctgaacaaagctccaagatccaaaagacagtcaagtctttcagattcatctgagaatgttattcatatctatcagcggaactatattattgaattgatcaagcaatttgtttactgaacaatcacttttttcaatgaaattctgagaaaagagccaactccatactttgaagtaagcttcag

SEQ ID NO: 18 - DNA, 1054 bp, Cucumis sativus
ggagcgcattgtacaaagaaaatccatctctaatctttgagtggactacaagcatggcgatggcgtcccttctttcacccagcgctgtaatcctacgccctcactcattccgcttctcacaatcatcactctccaatggattctccattattcctatccgctcaacacttcgtgttttctgctctgccaatggcaacagcatccacacttctaacaaaaacccagttatttggcgagcggggtcaacagacgagaaattatgctagggattggattcactgcattttcatttcaagaagttgtttctaatgccctagctgagagtgttgtggttgctgaagattatcggacgtatacagacgaagcgaataagttcagcttggtgattcctcaagattggcaagtgggtaatggtgaaccgaatggattcaagtcggttacggcattttttcctcaagaaacttcaacttccaatgtcagtgttgtaatctcggggcttggtcctgattacacgaggatggaatcctttggcaaggttgaggaatttgctgatacattggtgagtggactggacagaagctggaaaaggccaccaggtgtggcggcgaaacttatcgactgtagatcatctaaagggatatattacatagagtacacactgcagaatccaggtgaaagccgcaaacatttatactcagcaattgggatgtcatccaatggctggtacaatagactttacaccataacaggacagtatgcagatgaagaatcggagagctatagctccaaaatcgagaaggttgtcaattccttcgctttcatttgatgattgccacagaattggcctccaccacactatcataatggttaaatgttttccacatctctctctaattatagttctcttttgttattattattattattattttttgtaatgagttctaaacataatattgaattgtctttgatgcatctatatttttacattttcacgaggaatgaattcacatttctattaattcataaaagaatccacaaaacagaaaaaaaa

SEQ ID NO: 19 - DNA, 795 bp, Ricinus communis
atggcttcaatttctttactctgttgcaattgctacttcacatctttctccaacaagacacctctccatcttttgaaacctaacttaaacttcctctctgcttcaccttcttttcgatttaacagttgcagaaagcaacatcttccatgttgcaccaactctttcccagacgaagaccaacaccaaccattattctgtcgttttaggcttcaagaaccatatggaagaagagaagctttgttcagcgtggcatttaccactgggtttacttttccagggcttatttctaatgcatttgcagagattgatgacttccgcctttatactgatgatgccaacaagttccaaatatcgattccccaagactggagagtaggtgctggagaacctaatgggttcaaatcagtgaccgctttctacccagaagaagcttcaggctctagtgtcagtgtagtgatcacaggactcggtccggattttactagaatggagtcttttggcaaagtggaagccttcgccgaaactctggttagtggattggacagaagctggcaaaggcccccaggcgttgcagcaaaacttatcgactgtaaagcgactaaagggatttactacattgagtacacattacaaaacccaggcgaaggtcgcaaacatctgttttctgctcttgggatggctttcaatggttggtataacagactgtatacagtgacagggcagtttgtggaagaggagtcagagaattatggatcaaaggttcagaaggttgtttcatcattcaagttcatctga

SEQ ID NO: 20 - DNA, 1028 bp, Vitis vinifera
caatcaaaaaaagcatggctctgtattttccacttcctctccgttctgggtcctgcgacttctcagcttattcgagtaaaaaaggttatgggtcaagaaccgggaaatgtggaaaaaagcaacgtgttgtcttctgcaagaatgagaacaaggaagaagaaaaaacaagttttgggattaaagaacaacatggaggtggaagaagggaggttgtgctacagatggtgttcagtacaatttcccttcaggcaattgttcctaacgcactggccgatactgaggtgccagaggatttcaaggtttactcagatgaggtcaacaagttcaaaatacagattccccaagattggcaggtgggttcaggagaaccaagtggatttaaatcagtgacagcattctacccagaagaagcttctggttcaaatgtcagcgtagttatcactgggcttggcgcggattttaccagactcgagtcttttggcaaagttgatgcttttgcagagaatctggtaaatggattggatagaagctggcaaaggccccctggtattgctgcaaaactcattgactgcagagctgctaatgggttttattacattgagtattggcttcagaatcctggggaaagtcgtagacatttattttcagctgttgggatggcaaacaacggttggtacaacaggctttatactgtgaccggacagtatttggaagaagaatcagaaaaattcagttctaaaattgagaaggttgttgcatccttcaggtttatttgaagaaaaatttgcatgttcaggatataaactgaggctgaagattactggttcagcaactctgtggatttcacaatgcacacgaattggcattgtgcaaaaagatgagatgatttatatactcagattgcatcaggtgtcttttgttgtaaaattgtaaggaaggggaagggaaattatctctatgctaccattgaaaattttttccacacctttgcagttgcttcacattcatttgcagaattgatggatgag

SEQ ID NO: 21 - DNA, 726 bp, Medicago truncatula
atggcatccatttcatggttcagctgtctacacatccgaccaacagccactgccggcgacaaaggtttatcatctcccataaccgtggaacatcataaaacaagaccacaaaatttactctcatcctcggaagaaggacttgcgattaatagaagacaactaattctttacacatccactgcagcaattgcagcttcatctactgactcaaatgcattggcactcaatgatgtatctgaggattttagtatctacactgatgatgagaacaagttcaagatagatattccacaagagtggcaaattggaacaggagagtctgcagggttcaaatcattaactgctttctacccaaaagagcaatctaattccaatgtgagcgttgtgatcacaggagtgggtccagatttcactaagatggaatcattcggcaaagttgaagaatttgctgacactctggttagtgggttggatagaagctggaaaaaaccacctggtgtggctgctaaactcatagattgtaaatcatctaaaggattttatttcattgagtatacgctgcaaagtcctggtgagggtcgcaaacatctatattcagctattgggatgttaacaaatggctggtataacagactgtatacagtgacaggacagtatggggaagaggaaacagacaagtatgcttccaaaattcagaaggcagttcgatcgtttaagttcatataa

SEQ ID NO: 22 - DNA, 579 bp, Populus trichocarpa
ggaactaaaagaagagaagctttattcaatatggtatttactgcttttactttccctgcaattgcctctactgcattggcagccacaggcgtggcagaggattcacgtgtttataccgatgatgcgaacaagtttaagatatctattccccaaggctggcaagtaggtgcaggagaaccaagtggatacaaatccgtcactgctttctatccagaagaagcttctaattcaagtgtcagcgttgtgatcaccgggcttggtccagattttactagattggaatcatttggcaaagttgatgcctttgctgagactctggtgggtggattggacaggagctggcagaggcccccgggcgtggcagcaaaacttatagactctaaagctgctaatgggctttactacatcgagtatacgctgcaaaatccaggcgaaagtcgcagacatttgctttcagcacttggagttacattcaatggttggtacaacagactatatacggtgacagggcagtttgtcgatgaagaatcagagaaattcggcaccgagatcaggaaggtatatcagaactcttcattt

SEQ ID NO: 23 - DNA, 951 bp, Lotus japonicus
ggaatggcgtccatttcctggtcttgttgtctgcgttggcgaccaacaatatccgaccgcacagcctctgcggccgacaaaggtttctcacctcccataacattggagcatcataaaaaaacaccatgtttactatcagcacgcaattcctccattgaagaaggacatgcggttaacagaagacaacttgttttctacacgtcactagctgcatttgcagctgccccatctactgtcctgaaggcattggcactcaatgatgtggttgaggatgttcgtatctacattgatgatgagaacaagttcaagatagagattccccaagattgggaagtaggaacaggagactctagtgggttcaaatcattaactgcattctaccccaaagaggcatctagttccaatgtgagtgttgctatcacagggttggggccggatttcactaagatggagtcgtttggcaaggttgatgagtttgctgagactctggttagtgggctggacagaagctggagaaaaccgcctggtgtagctgctaaactcataaatagtaaaccatctaaaggaatttattatatcgagtactcgttgcaaaatcctggtgagagtcgcagacatctatattcagctatagggatggcaacaaatggttggtataacagactgtatactgtgacaggacagtatgtggaagaggaaacagacaagtatgcttccgaaattcagaaggcggtcacatcatttaagttcatataaagaaatgctcatgatgaaggagaaatttccccacagccatctttcctatataaatacagatttgtgccttcctacagtgtaggattcttatgagcaagagaggattcttatatttgtctttatgagcaaaatggaatacttcattatttcattcctctcttatgtctcttgctcctcagattatgtatattgtat

SEQ ID NO: 24 - DNA, 866 bp, Fragaria vesca
atggcttctgttgcgtcttggcatcctctgttccttcgacctcgcacatcccatttcaccacgacctcctacaacacaggcaccgccatatgtagaaagagctatctgcaatgttgcaacaacaaagaacaagaaccacaaccagaacaagaagaaaaatcggtttttgggatgcaatgccaagccaagagaagacaagttttgcttgggactacttttgctgcattttcttttccggaaatttattccaacattgcattggccgagaatgacgattttcgtgttttcaccgatgatgtcaacaagttccagatatcaattcccctagactggcaagtaggcgcaggggaaccaagtgggttcaagtcagttactgctttttacccggaagagggatctagctcaattagtgtcgtaatcacggggcttggtccggattttacgaagatggaatcctttggcaaagttgacgaattcgctgagactctggtcagtggactagataggagctggcaaaggacagcaggagttgcagcaaaactcatagattgcaaatcatctaaagggatttactacattgagtattcgctacagaaacctggtgaaagtatcaagcacctctattcagctcttgggatggcaaacaacggctggtacaacagactatataccgtcactggccagtttggagaggaggaagcggataaatacagatccaaaattgagaaggctgtaaaatccttcaagttcatatgataaacaacctccagaggggcagagtttgaattgtgaactacggtttaccaattttgattgggtcagttgtacacaaatttttcatcgtaatctaatgtaatacatttgaa

SEQ ID NO: 25 - DNA, 1015 bp, Glycine max
gtgaataataatcagaacaaaaccaaccatttaaaaaaaaaaaaaaaagaaatggtggcagagaagctgatctgaaaggaatggcgttcatttggcggttctgtggtgtgtctctatgcaacttcacagcctctaatgcccagaaaggtccttctccttctctgcccataaccttggacttggagcatcatataacaaccccatctttactttcttccatcgaagaagaagaaggacgcgcggttaataggagacaacttattcttcacacgccagtagctgcagcagctgcatttgcagtcccaaatgcattggcactcaatgatgtgtctgaggatgttcgtgtctacactgacgatgagaacaagttcaagattgagattcccgaagagtggcaagtgggaacaggagacggagaatctagtgggtttaaatccataactgctttctacccaacacaggcatccaattccaatgtgagcgttgtgatcacagggctgggaccggatttcaccaggatggaatcctttggcaaagttgacgagtttgctcagactctagttagtgggcttgacagaagctggcgaaaacccccgggtgtggctgctaaactcatagattgtaaatcatctaatgggatttattacatcgagtatttgctgcaaaatcctggtgagagtcgcaggtatttgtattcagctattgggatggcatcaaatggttggtataacagactgtataccgtgacaggacagtatgtggaagaggacacagacaagtatgcttcaaaagttcagaaggtagttgcatcatttaggttcatatgaagaaaatggtcatgacgaggaagaatttttatcacagcacttcatctattctatttcattatggattttcctggcattgttctttaagctagatatggcattctagatcggactggtatgataaaaaccatgacatttccttcgagattgttgaatgaaagtaatatacttagtggccataattgaca

SEQ ID NO: 26 - DNA, 1159 bp, Solanum lycopersicum
ggctgtgaattggatacaccaatatctctgcttcttcaaagaaaacaaaaaaaataaaaacagaaatggcgactctttcatcttcatcttcatcttcatcttcatcttcatctccatgtttgaaccagtaccagtatcaagctattcttcgcttgccacgtgtccctttaatttcctctcatcttcttaaagttcccaagaaaaatcgaaactcacttattttctgctgcaacaacactgtgcctgattcaagaacaggtgagcaagttaaaggagaatgcttaaccaagagaagagagctcctgctacaggcaggctctgttgcattttctctgtccgcctttacatcgattgcattggcagagaaggatgtcccggaggagtttcgtgtttattcagatgatgtcaacaagtttaagatcatgatacctagtgattggcaaataggcgcgggagaaggtgatggagtaaggtcactcttagctttctatcctccagaagcttctaactcaaatgtcagcatagtaatcacaagccttggtgctgatttcaccaagttggaatctttcgggaaagttgatgcttttgctgagaatctggtcagcggatttgatagaagctggcaaaggcctccgggagtgaaagcaaaactcatagatagcaaagcttctaaagggttgtattacatcgagtacactctccaaaatcccggtgaaagtctcagacatctattttcagtgcttgggatagcaaacaatgggatttacaacagactgtatactctcactggacagtttgtagacgaggaggcagagaaatatggtgccaaaatacagaaggctgtttcttctttcagattaatatgatgacatgaacagagagcgcgatatcgcaaattttggcttgagcttctggtttttctcgtttggtgaatggtaaacataattgagagcgcgatatcacagattcaagttctggttaaggtatattatgacgactcgagaaaaaactggagttgtaagtatgaactagcaacttgatcaatgttagagttagtatttgcatatatcgttatataccaaaactgtatcgattttttgataaaaatatgaccttagtgcaaataatttgatgctcaagttttgattatatatttgta

SEQ ID NO: 27 - DNA, 1680 bp, Cicer arietinum
tctcgtaaaagaatgagattcagttgaagttatcgaagaagaagaatgcagcagaggaaaaggcaaagtatggatgggcctagcatctatgcgtggttgttttgtgtcattggaatgacatcacttttcggtgctgctttcctaccaccagatatagggattgtgttttttctcagacaaatatgtctgtttgtgtttcgatctatgtggatgacaaggttggtgttttttctagctgcagctgcacatgtcattgaggctatctatgcttggtgcttggctagaagactggatccttccaattcaagggcttggttttggcaaacattggctctaggctttttttcattgcgttttctattgaaattgaaaagatcaaaggaataactttgaaataatcacttcttgtaccattgttattttcagaaatcaattatctttcccatcaattgtatgccttttttttatgtaaaattaatatttttacaagttgttattagttatcactgtcgaataaatttaccatgacagtacatatcttttaattttgaaaattgtccattttgttttcttatctataatggttttcttctctatttaattttggatttaattaaattagaaatagtgtcttctctgtggaggataaaagtgtaattaaatagataataataataaaggaaatgaagggtgagaaagagaagctgatctaaaaaggaatggcatcaatttcatggttcagctgtttacacattccaccaacatcctctgctgccgataaaggtttatcatcatctcccataaccgtggaacatcataaaacaacaacacgtttaatctcttcctttgaaggacaacaacatgttgttaatagaagacaactgattctttatacatccacagcagcaattgcagcactatctactgtcccaaatgcattggcactaaatgatgtgtctgaggatgttagtatctacactgatgatgagaacaagttcaagatagaaattcctcaagagtggcagataggaacaggagagtctgcagggtttaaatccttaactgctttctacccaaaagatgaatctaattccaacgtgagcgttgtgatcacaggggtcggaccggatttcactaagatggaatcattcggcaaagttgaagaatttgctgacactctggtaagtgggcttgacagaagctggaaaagaccccctggtgtggctgctaaactcataaattgtaaatcatctaaaggattttattacattgagtatacgctgcaaaatcccggcgagagtcgcaagcatctatattcagttattgggatgtcaacagttggctggtataacagactgtatactgtgacaggacagtttgtggaagaggaaacagaaaagtatgcttccaaaattttgaaggcggttgcatcgtttaagttcatataaagaaatgcttgtgacgggagagaaatgttctcattggtttctttcatgggctgccgtttaatgttttcatgacattttttgtaagctagaaatggcgtctaaatgttataaatatgatatttgctatggtacttccttcaaaaactgataaaccagagtaggctaaatgaatggcacaaattgatgtaatggataagatattttgcagtgaatatcagcaccttcagttaaa

SEQ ID NO: 28 - DNA, 1068 bp, Triticum aestivum
gaagcacagcagcgtcgtcgaccaccatcgagccgtactccatggctgccgtgaccaccgcctctctctgtcccggcctcggcaagccccgccgagaccacgcgaagccaccgagaaccacggtctgccattgcctccctgctcggaggacggaggagggggtgaagcggcgggacgccctgctcggcgtcctcctctccgctaccgccgcgtcgtcggcgccgctgctcgtccccgccgaggctttcgccgaggtcgccgatgcgcaggaggggttcaccgcgtacgaggacgaggccaacaagttcaccctcgtgattccacaaggctggcaggtcggcgcaggtgaacgcagcggcttcaagaacgtgacagcgttcttccccgagcaaaaccccaactccagcgtcagcgtcgtgatcaccgggatcgggccggacttcaccagcctcaagtccttcggtaacgtcgacgagttcgccgaaaacctggtgaccggcctggacaggagctggcagaggccggcggggctcgcagcgaagctcatcgactccaaggcatcaaacggcttgtactacatcgagtacacgctgcagaaccccggcgagaagcgccgccacatcgtctccgccatcgggatggcattcaacggctggtacaatcggctgtacacggtgacagggcagtacatcgacgacgacgaggagtcagccatatacaaacctgagatagagaagtctgtcaagtcgttcaagttcacatgaaatgcccccaaaaaggaagttcaggtgagaacaagtatagagtgacagagaagagagagtatacaaagctagtagctcctgatgtcaagttcaattagtgagtatgcatatgtttgtcgaatttaccggaaagaaaagatgaacaccagatgttcgaagacttcgatggcgtagcttggctgagaacagcattggcagcatgagtgtgagatagagcatgagtgtcgttggttctaagaaaattgctagaactctgttacaaggaaactaaaattgctctgatgtaaaaaaaaaaaaaaaacga

SEQ ID NO: 29 - DNA, 1037 bp, Oryza sativa
gcaaggcaggcagcagcgaccagacgaagcagagagagcgcccgcgccgcgccggccatggctgccgccgtgaccaccaccaccaccgccacaaccacccatctctgccgtggcctctcctcctcctccgccgccgccgccaagccgcggcgagcgacgacgctcagatgcggcgccgctgctcgggtggaagggctggggcggagggaggcgttgctcggcgtgctcctctccacggcgacggcggcgtccgcgcccgtcgccgccgtggccgcgaccgccgagttgcaggaggggttccgcacgtacgaggatgaggccaacaagttcagcatcgccattccacaagactggctgatcggcgccggcgaggtcagcggcttcaagtccgtcacggcgttctaccctgaccaagtcgccgactccaatgtcagcgtagccatcaccggaatcggccccgatttcaccagcctcaagtcgttcggcgacgtcgacgccttcgcagagaccctggtgaacggcctggacaggagctggaaacggccgccgggggtcgccgcgaagctcatcaactccagggcagccaacgggttttactacatcgagtacacgctgcagaaccccggcgagcagcgccggcacattgtctcggccatcgggatggcgttcaacggctggtacaaccggctctacacggtgacaggccagtacatcgatgaggacggggatgtagacaagtacagggctcagatagagaagtgtgttcagtcattcaggttcacatgaaagaggagcatcctacacaacatccaacaaggcgaggacgaaaaacattttgtaaaccaacgtatttcgttataattgtaaatcaatcagtatattcatgtcatcagttcaaccaactaaatgtacaccaattgttccgagattttgacgatgcggccttgccgaggccaacatgagctaattatgttgtggcaagtcataagcattgttttctatgcatttttaagggagaaaaaacaggtgtatttgtt

SEQ ID NO: 30 - DNA, 1269 bp, Brachypodium distachyon
atggcccggctcggcccggcccacgtgttttacagccgttgggctgggccgtactgccaaaacgtgtccaaatggcccacgtcgaagacgaactctcacgggccgacgtccttggcgcgcggccatggcccatgggtaagtaagatacgagggggccgaagcaatgtgcggcggaagttcccggacgacgacacgacggccggccaccgtacaaagcttctcagcaaaatatcctccccctcgaaagccaccagcgcagcagcagcgcagagccattcgctcgccatggctgccgtgaccaccgcctcctccgccatctgccccggcttcagcagcaacccccgccgaggccacgcgaagccgcggagatccacggcctgggcctgccattgccgccgctcccctgccctgcgcgagcaacaacctacggcggccgttgccgggacggcggaggaggggctcaggcggagggatgccctgctcggcgtcgtcttctcggccggcacggcgacgctgctcgctagtcccgccggtgctctcgccgaggccgctgccgaggtgcaggaggggttcagcgagtaccaggacgaggccaacaagttcagcatcgtggttccgcaaggatggcagatgggcgctggtgagggcagcggcttcaagaacgtcacggcgttcttcccggacaaggccgccgactcgagcgttagcgtggtcatcaccgggatcgggccggacttcaccagcctcaagtccttcggcgacgtcgacgccttcgccgagaacctggtgaccgggctggacaggagctggcagcggcctgcgggggtcaccgcgaagctcatcgactccagggcgtccaacggcatgtactacatcgagtacacactgcagaaccccggcgataagcgccggcacatcgtctccgccatcggcatggcgttcaacggctggtacaaccggctctacacggtgacagggcagtacatcgaagatgacgaggagtccgtcaagttcaagcctcagattgagaagtctgtcaaatcattcaagttcacatgaaatgccttcaaaacaaaggtcacatgaaaataagtactgctactacttttgaatgaagtactatatctaagcagagaagagaaggtatataaaggcagcttccggtaatgtgtgcagaacgaaatgaactaaacctttgtgaatgtaagggttgtgagctttgagaatatatatgtttgtcaattttactgaatacatagctctagactt

SEQ ID NO: 31 - DNA, 1024 bp, Phyllostachys edulis
atagtgccatacgccatggccgccgtaactaccgcctccctctttcctggcctctcctcctgcagccccaagcccagaagccacaggaagctgcagagaacgacggtctgccaatgccgccctgctcggatggaggggatgaaacggagggaggccttgcttagcatcctcctctccactgccgcttcggcgccgccgcttgctcctgccgaagctttggccgagaccaccgagttgcaggagggcttccgtacgtacgaggacgaggctaacaagtttagcattgcggttccacaagactggatggtcggcgcaggcgagggcagcggcttcaagtccgtcacggcgttctaccctgaaggcgccgactcgagcgtcagcgtcgtgatcaccggaatcggaccggatttcaccagcctcaagtccttcggcgacgtcgacgccttcgccgagagcctggtgaacggcctggacaggagctggcagaggccgccggggctcgccgcgaagctcatcgactccagggcagcgaacggtctgtactacgtcgagtacacgctgcagaaccccggcgaaaagcggcggcatatcgtctcggccgtcgggatggcgttcaacggctggtacaacaggctctacacggtgacagggcagtacatcgatgacgacgacgagccaggcaagtacaagcctcagatagagaagtctgtcctatcgttcaggttcacatgaaagaactaaactacagtctacccagagtgcaacaatatgcagagaagataaagtagataaaagcccttccgcagataagttcagaacggaagatacgttgtgatttttgtcaatcagtgagcatatgtttgtcgatttgaccaaataaaatatgtactccacatgttcgacgacttgctgtgcccagcatgagttaattgtaagagaagttaccatgcgccggacctgtcattctgaaactgtgatgagtgacattctgaaactgtaacatagtaaacgtatgttcagtttt

SEQ ID NO: 32 - DNA, 1053 bp, Hordeum vulgare
agagccgtactccatggccgccgtgaccaccgcctccctctgcccgggcctcggcaagacccaacgaggccacgcgaagccgccgagaacaacggtctgccattgcctccctgctcggaggacggaggagggggtgaagcggcgggacgccctgctcggcgtcctcctctccgctaccgccgcgtcgtcggcgccactgctcgtccccgccgaggctttcgccgaggccgccgaggcgcaggaggggttcaccgcgtacgaggatgaggccaacaagttcaccctcgcgattccacaaggctggcaggtcggcgcaggtgaacgcagcggcttcaagaacgtgacggcgttcttccccgagcaaaaccccaactcgagtgtcagcgtcgtgatcaccggaatcgggccagacttcaccagcctcaagtccttcggtaatgtcgacgagttcgccgagaacctggtgacaggcctggacaggagctggcagcggccggcggggctcaccgcgaagctcatcgactccaaggcagcaaacggtctctactacatcgagtacacgctgcagaaccccggcgagaagcgccgccacatcgtgtccgccatcgggatggcgttcaacggctggtacaaccggctctacacggtgacaggacagtacatcgatgacgacgaggattcagccatatacaagcctgagatagagaagtctgtcaagtctttcaagttcacatgaaatgcctccaaaaaggaagttcaggtgagaacaagtatagaggaacagagaagagaaagtatacaaaactggtagctcttcatgttaagttcaattagtgagtgtgtatatgtttgtcgaatttaccggaagaaaatatgaacaccaaatgttcaaagacttcgatggcgttgcttggctgaggacagcaatggcagcatgagggtatgagatagagcatgagaatgtcgtttgttctgagaacattgctagaactccttataagaaactaaaattgctccgatgtaaacttcttcctagcatctatttttgggctc

SEQ ID NO: 33 - DNA, 1138 bp, Zea mays
cccgttgccacacatacggatccaacaaaatctcccgcaaagacaacggcgagccaaccaccaccagcgtcccgcgctagctgcggcaccgcatggctgccgtgaccagcaccgcctccatctgcccggccgcagccggcgccctctcttcgctgccgtccttcatcacgcgcaagcccaccagcggcagcaggaggttgcagcaggcagcagcgacgacagtctgccactgccgctctgctcgggtagaggaggggctgctgggccggagggacgccttattgctcggcatcgtcttctccgccgcgacgccgccgctgctcgcccctgccggcgctctggcggacgaggccaccgccgagtcgcaggagggcttcactacgtacgaggatgaggccaacaagttcagcattcaagttccgcaaggctggctggtcggcgccggcgaggccagcggcatcaagtctgtcacggcgttctaccccgagcaggccgccaccgactccaatgtcagcgtcgccatcaccgggatcgggccggacttcaccagcctcaagtccttcggcgacgtcgatgccttcgccgagggtctggtgaacggcctggacaggagctggcagaggccgccggggctcgccgccaagctcatcgactccagggcggcaaacggcctgtactacctggagtacacgctgcagaaccccggcgagcgacggcgccacatcgtctcggccatcgggatggccttcaacggctggtacaaccgcctctacactgtgacgggccagtacatcgacgacgatgactcggagaagtacaggcctcagatagagaaggctgttggatcgttcaggctgacatgaaagatgcgatgtcatccagcaccagcagcagcagccgcccacggtacataaaccctaaatatgtatgcggagaggtccagcaacatgttgtgcccgaaaattgacaccttgccatttcgatgagacaagacaaggcatgtgcctattgccctattccaattcttgagcactgtaacactgccaatatgcagagtatatgttttctgcctgttgaggtggatacaaatgcatgcttttttttttattaataactcatgtgtaacactgctgccttt

SEQ ID NO: 34 - DNA, 1162 bp, Sorghum bicolor
agcgcgagcctgccagccaaccaccgccaccggctttcatcccgcgcgtgcgtcctgcgctagctgcgcccatggctgccgtgaccagcaccgcctccctctgcccggccgcagccggcggcctctctgcctcgtcgtcgtcgccgttcacgcgcaagcccagcagcagcaggaggctgcaggcagcgtccacggcctgccactgccgccctgctcgggtagtagaggggctggaccggagggacgccttgctcggcatcgtcctctccgccgcggtggcgccgctgctcgcccctgccggtgctctagcggacgagcccaccaccgagtcgcaggagggcttcactacgtacgaagatgaggccaacaagttcagcattcaagttccacagggctggctggtcggcgccggcgaggccagcggcatcaagtcggtcacggcgttctacccggagcaggcagccgccgattccaacgtcagcgtcgccatcaccgggatcgggccggacttcaccagcctcaagtccttcggcgacgtcgactccttcgccgagggccttgtgaacggcctggacaggagctggcagaggccgccggggctcgccgccaagctcatcgactccagggcggcaaacggtttgtactacctggagtacacgctgcagaaccccggcgagcggcggcggcacatcgtctcggccatcgggatggcgttcaacggctggtacaaccgcctctacacggtgacaggccagtacatcgacgacgatgacgattccgaaaagtacaggcctcagatagagaaggctgttcgatcgttcaggctgacatgaaagatgccatgtcattcagcagaggtcttgtgcctgaaaattgacaccttgccatttccatgagatgagacaagacaagacatgtatgccaattcttgagcactgtaacactgcaagtatgcgaatatattttctcctttttgaggtggatataaatatgttttttgtaactcttgtgtaacgttgctgcggtgtttttttggttgtgtatatgtaatgtttagagggtcgggctgaaggagcaactatgtgacctttattctctttttaaggcaaagttcgtgtcacttcttttcaaaacaagcaaatggttttgtttcttgagctgg

SEQ ID NO: 35 - DNA, 1062 bp, Setaria italica
cggtgcctaccaaaacacacggctggaacaaaatatcccccacgaaaacaaacggcgagccaaccgcaaccaccactcggcaccggctggcctgcggcgcgcgccatggctgccgtgaccagcaccgccttcctctgcccggccgccggcggcctctccccctcgccgcccttcaggcgcaatcccggcagcagcagcagccgcaggaggctgcagctgcaggtctgccactgccgccctgctcgggtagaggggctggaccggagggaggccttgctcggcgtcgccctctccgccgccgcgccggcgctcttcgcccccgcggctgctctggcggccgaggccaccggtactttgcaggagggcttcaccacgtacgaggatgaggccaacaagttcagcattgtggttccacaaggctggctgatcggcgccggcgagtccagcggcatcaagtccgtcacggcgttctaccccgagcaggccgccgactccaacgtcagcgtcgcgatcaccggcatcgggccggacttcaccagcctcaagtccttcggcgatgtcgacgccttcgccgagggcctggtgaacggcctggacaggagctggcagaggccgccggggctcgccgcgaagctcatcgattccaaggcggcaaacggtctgtactacgtggagtacacgctgcagaaccccggcgagcggcggcggcacatcctctctgcaatcgggatggcgttcaacggctggtacaaccgcctctacacggtgacaggccagtacatcgacgacgaggagtcggagaagttcaggcctcagattgagaaggcggttcgatcgttcaggctgacatgagagtgcttcgcactgtgtagcattcagagatgcacggtatgcaggtggacgcctgtaaattgaccaactcgtcttccacattattaagtttttttttaagcaagtctcacggtatgttggaaagtacattgctacacctcaacaatcccatagatcgtctcatgtaatgccacatataatttttgctggtgtggaggaaggagggtgatg

SEQ ID NO: 36 - DNA, 1091 bp, Picea glauca
acttcaaaatcccaaacccatcagaggagggagttccaacagatgactatcgtggtgaagatgggcatgcttggcctggtgtcatcaccatcaattcccactactcacaatctatgctctccagtccaaccattcagaaggaatttcaagaatttcaagcaggggaaaaagcaagtcacaggctgtttcgaaatccagaacaatctgtcctcccatgaattgtcaagaaatggaagaaggcaggccatatgtcagattgctgctttgttctcagcgattccttgtactgtttcagcggcaagggcagcagaaactgagcttcaagaagattacgagttgtataaggacgagacagacaaattttcactactagttcctcgagactggataaagggtgaaggaaaaacagatggacagagagcagtgactgccttctaccctgaaagcggcatagtttctaatgtgaatgtaataataacaggactttctgctgactatacaaaaatggaatcatttggcactgttgatgcatttgctgagaccctggttaattctctagatagaagctggaaaagaccgccagggcaagcagcaaagctgcttaatgcaaaatccaaaaacggcttgtattatatagagtattcattgcaaaagcctggggagagtaagatccatcttctctctgcgatcggaatggcaatgaatggttggtacaacaggctttacactgtaacggggcagtatctagaagacgatgctggcaaatatggctcaaagattgaaaagtccatttcatctttcagattagtttgaaagattaattaccttccatgtgaggcatcaagtatgttgggaaaagacttataatatacaagagcataaaggtgataaatattaaataattaaaaatcccccattttattcatcttcaattatgtctggaataaacttgatttaccttgtaatatataatgtatgacctaatatcttatttggaactaagtgtgaaaccactcatagttattccaactaaattttagtttagacaagggaataaaatacattcaatgtccttattgtttactaaaaaa

SEQ ID NO: 37 - DNA, 355 bp, Arachis diogoi
ggggtgggtccggattttactaagatggaatcgtttggtaaagtggaagaatttgccgagactctgattggtggattggacagaagctggcaaagaccaccgggtgtggctgccaaactcatagattgtaaatcatccaaggggttttattacatagagtattcactgcaaaatccgggtgagagtcgcagaaccttatattctgctattggaatggcatcaaatggttggtataacagactctacacggtgacaggacagtttgtagaagaggaaactgacaagtatgcttccaaagtgaaaaaggctgttgcatcatttaggttcatatgaacaaagagttcatgagggagat

SEQ ID NO: 38 - DNA, 1089 bp, Physcomitrella patens
gcaggagcaatggacgctgtcgttggtcgcacctcatgccccttgtctctgtcttcctcgtatcaatggattgctgggtcgccatctgcttctcgtgctacagtcgttgttagaggtacaagccggcgtgacggtaaacacaaagcagtgcgttgcgagcaggttccagaatgcagcaccagcaattgtcaaacaatgcagagacgagaggttatcggtcaagctctattagccatgtccatgagctttgctcctccagctcgttcggccacagacacagatgctgctactgaatttacgacttacgaggatgcagccgataaattcacattgctcgtgccacaagcctggaacagaggcgaagggaaaacgtccgggcaaaggaaagtcacggctttctatcctgcggatggcggtcttaccaatgtaaatatagtcataacaggactcggagcagatttcacgagtttaggatcctttggcacggccgacaatttcgcggagaatttggtgaacagtttggacaggagttggcagaaacccccgggccagaaagcaaggcttgtggattgtaaatcaagagcagataaatactatgtagaatacactatacagagactcggagagcagcagcggcacttagtctcagttgttgggattggaaacaatggatgggtcaacagattatacaccgtcacgggccagtactttgaggaagactcagccaaatataaacaagacattaacaagatcatctcctctttcaaaatactgtagttcatagatcgaagactcggggcacagactgcagaccatggagtttatgactgaccagcattgtggtaaaacctgggattttcgttcctcatgcttcgtgtcacagagaagctcattgagttgggagaactgaagtggttgtgtaaacacgctggggttgttttgcatgtggtgagagcagatgtccttcgagcagccattcataaatctcaagatgagtttattctgttctgcagaaactgccgaacctggattcttgtaatagaaccattcaataatttccaaggtcaccattgggcctgagatatcatc

SEQ ID NO: 39 - DNA, 2425 bp, Selaginella moellendorffii
atgggggaggagaagcgcgagaatctcatggagtcgctcttcggggaggagtcggatgacgacgccgatgccgctgcctcctactctgaggaggagggcgaaggcgaaggcgaggcagagggcggtggtgccgagagcggtggcgacagggaagagagcgagggcgagcgggaagccagtgagggcgacaaggaggagagcgagcatgagagagtgtccaggaggagcagtgatgacggaggtggtgaagaagggagcgccgccagcggctctgagaacgatggacaagtccaggaaagggaagcaactcgcagcgaggaggtggaggagcagcgtggtgctagaattcgtgcagcattgggtgattctgatgacgacgatcaggaggaaggaggagttgacggccctcgcaagccatcgagtccagagggggagggctcggacttggagggaagctaccacaaagatagtaagcggggtgcagaggatgacgaggagcagtattactctgatgaagagcgcgcagaaatcaagaaacccaagggtgaacctcttacagtagaagttccactcaggcaacctccaactcaggctcacaacgcaagtagtttggcacttgtttctttttcattatctcgtgagcttacgggcctttgctttcagatgaatctcgtcaggatctccaacattatggatatagagcaaaggccttttgatccaaagacatacgtcgaagaggatggatttgttgatgaaactggccgacgccgtatacgtatagaggagaacgtggtgcgctggagatacgtcaggaatcgggatggctcgcgctcggccgagagcaacgcccggtttgtgaagtggtccgatggtagcatgcaacttcttctcggcaatgaagttctggatcttgctgttcaagatgggcaacaagacgaatcacacttgtttatccgtcagcccaagggattattacaagcccaagggaggctggcacgtaagatgagattcatgccttcgtcgttgagatcgaagtcgcaccgtctcttaactgctctcgtggattctacgcacaagaaggtgttcaaagtgaagaatgtgatcacggacttcgatcccgagaaggacaaagaacaaaaagagaaggcagcagaacagaggattaaaagcaaagaagatctccaaaaaaagcaggagaagacgatgcgtaaatacccccctacacgggagagagaacctcagctttctcctggataccttgaaggggcgcttgaagaggaggatgaagattatgacgacgaggggcgtagcaaccgacggtaccaagaccagcttgatgccgaaagcagggcggagagacgaatcaaccaggttaagcggcaaccaccaaaggcaatggagcgacgcccttcttcgcggagcaggagggatattttggaagacgaggattcagacgagagcgaccgcaatagaggtgcgcgaggtgatgaaggtgaggaagagcaggaagatgacgagggggaggaagaagaggaggaagtggaggcaagggatagccgccgcaagaggaaagacagggacagggaacagctgcagcagcagcaaaattcgcctcccagaaagcagcaaacgcacaggcggagagcagtagtttggtttctcgccacaggttgcaagagtagaatagataggggcagccagggaagtgtggcgtcatggcaagtgtgcatacaaactgctatgttcgtccagcagttccagccagttcaagtcgaccgccattcaatgctcctgctactgctgcctgtccaccgctgagcaagagaaatctcttattgctggtgcctctgttggcgatgccggcgacgcctgtgtttgctgctggtattgtacttgtcaatcgttcgttaaactttgatgcaagacaggagcctcagatgaatatcaagtatacgaggaacaagacaagttctccctcactgtacccaaagactggataaaaggcgaggggaaagtcggatccagaagagtggtggcattccatccatccaaggctactttcccaaacgtgaacgtgatcatcacgaacctgggtgccgatttcaccgggatcggctcactgggatccgtggactcgttcgccgcgagcgtggttggcagcatggatagaagctacaagcggccgcctggaacagcggctcggctggtgaatgctgtgtcgagaaacggcatgtattatctcgactacaccgtccagacgcccggggaagcccagcgccatttcttctcggtggccggtgttggcgagacacagttttacaagcagctctacacggcaaccggccagtactgggaggctgatggagacagggacaggaaagcattgcaagaggcgatagagtcattccggattgttcacaagtga

SEQ ID NO: 40 - DNA, 832 bp, Camellia sinensis
  misc_feature (90)..(90): n is a, c, g, or t
atacccaaagttgccaagtggggccgggggaaataaaggagatcaagtcagtaacggagttgtacccgatgggacctctgatgaaagtcncgtggtaatcgcggcctggtgcgggttttaccagaatagaaatcttttggtaaagatgatgcttttgcagagaatctgctacgggctgggacaagaagctggcaaaggccaccggggggtaagagcaaaactcatagactctaaaactgctaatggtttgtattacattgaatatacactgcaaaatcctggccaaagttgcagacatttatttcagtgcttgggatccgaacaatggttggtatccagactatataccgtcactggacagtttgttgatgaggattcagaaaaatatggctccaaaattgagaaggctgtttcatcgttcagattaaactgagattttgaggatcctttccatttttgctttcaacatcggctctcatcgctgcaacatgtccaattgaagtcaagtttactaaaggaagcaaagcattgaatgatgtttgcatcctggccgaggatttccatgcacctggagccagctgtttggaagacaccaagaggcggctagattgtggcatatttactctctgttttacttttgttattcctagcctttcttgcaacttttcttgaagtatgctggaacctttattatttatttgactaggaaatttattcttaataccaccagaaagagatagacaaaaactaccttggtgattgcattgaattaacataaagtgcccaaaaatattttgctaagaaaaaaaaaaaaaaaaaaaaaaaaaaaaaa

SEQ ID NO: 41 - DNA, 2246 bp, Zea mays
tttggtgtttctcgcagtgcgcagagggcttcagtcattatcgtctcgtgctctctattgatggtagttttttgcttgggaagtataggggcacattgttggttgccatttcatgtgacgtggacaacgcattggttcttttggcatttgctttggtggtgagggagaacagagatagttcgttttggttcttgcgacttgttcggatccatgtcgtgggccctggtcgggagattggtgtcatatatgacagaaaccagggtattcttaatgtagtgcaagagcagattcctggctacacacccatgcaccacagatggagcactcgacacctagtagaaaatctttttcgaaagggttgtaccaagaataattcccccctttttgaggaggtctgtcgacagttggaggtttcgttattcgaggataagttgaaggaattaaaagatacaacaaatgatgaaggtgaaaaatggattgctagatttcctaactgtatttcctcgtctcctacacaaaaaacagtaagtacgaatgcaacattacgactgatgctatcaaaaagcaatatcaacctcatcgtaatctaccacatgtccaaaaataacccacaccaagatcagaaggaactaatccatacttagcttcattaaaaccgccactcattttttctttttctttgcctctggctcaggccaatgggacctaggaccatacaaccactctatgaaactacacttacgcccaccgtatggccgtaggggaataaattagtaaatttgtgaaaaaataacaaaattttggacatttgttatgcactcacataattactgttgggacacacgaagtacttcacagtgtccttacataagacaacacgatctccgcaatcacaccgaggcggagacttcagtcgtctttctgcgactaagttcttcttctcatccgtcattggtgtcgtgtcgggggaggaggcacccaacgcttaaaacactgtatattccttctggacaaccaattagcgaaaaggagatatcgatggtcaaatttatgaggaccgtcgatccattggaaaacacatcaagtgatcctacagaaatggaatgaagcattagtacacatgtagtaaacatcaataacacacaagtcataagctacatatgttaaaaacgccacaagtgtagaagcagcgagcagccgtgtctagatatttgaattgacatacccaaggcggtctgccacagtcacaattaggtacaggaagatcaggaggaacatgagcatccttactagatacatccagatacaactcccgaggacgatctctcttctgccacaacgactcctaatacatgtcttttcatctaacaaacgattatatattaacacaactatatagaaataacagaaatgattttaacttataaatacatgtatttcataaattatctaacaaactgtagtcattatatgaaccatatatcataggattcataactaatagcaatatgagcaacaatcaaaactaattaatcgaaaacatacaacgcaatatacgtaacaaatgaatcagtgagacactataccttggtcttcaaagttttccaactcgaatacgaagattggagcacctctgggtggtatggaagaagatacaaatggttgggtgcagctctcggctaggaaacaaccgatttataggccttcctagctcggcgccacagatccatggcgccgagctagtgccatgtcggtgctgcatcagccctcgacgctagcggccttgtgttaccttggtgctacaacttatgatattgagcaacgagtccaaatgcagaaataagttatctaggggtctaaacattaaacacgatttttttcttaaaaaggaccaacataaaaaaaactcgggctggcggcctgccagcgcccggggaccgtgagcccgtgaccccagcgggcccaaccagtcaaaaccgcaagagagagtcgtgaggcgtgcgcactaccccgagaaacgtgcgacgggaacctccgcggttccccaagttcgcctccttcactactctcgcgccccggcacgcctgaaaaaccccacccctcctgccgctccgcctctcccatcacttcccacgcccctcgccgcctcccattccagcgtggacacgacgccactcgccagcacggagacgcgcgcctcgaagcactactgcactagccagccgtcgttcttccgcgccggcgcc

SEQ ID NO: 42 - DNA, 27 bp, Artificial
  synthetic
tttttaggaattattgagtattattga

SEQ ID NO: 43 - DNA, 24 bp, Artificial
  synthetic
aaataaaaatcatacccacatccc

SEQ ID NO: 44 - DNA, 26 bp, Artificial
  synthetic
tgttgaattattaagatatttaagat

SEQ ID NO: 45 - DNA, 25 bp, Artificial
  synthetic
tcaaccaataaaaattaccatctac

SEQ ID NO: 46 - DNA, 30 bp, Artificial
  synthetic
taagttttttttaagagtttgtatttgtat

SEQ ID NO: 47 - DNA, 25 bp, Artificial
  synthetic
taaaaataatcaaaacctaacttac

SEQ ID NO: 48 - DNA, 25 bp, Artificial
  synthetic
attgtttattaaatgttttttagtt

SEQ ID NO: 49 - DNA, 24 bp, Artificial
  synthetic
ctaacaattcccaaaacccttatc

SEQ ID NO: 50 - DNA, 24 bp, Artificial
  synthetic
gtgtactcatctggatctgtattg

SEQ ID NO: 51 - DNA, 25 bp, Artificial
  synthetic
ggttgaggagcctgaatctctgaac

SEQ ID NO: 52 - DNA, 1000 bp, Arabidopsis thaliana
acagaaaaaaaaaaactaatttcgattccacaatgccgaaacccagaaaaattctcaaaacgaagtcactcaagaagataatcaacaaagcgaaaacggagaagggtttgggtttaaggtaccgtaacgaactccggtaagttccgatgatggtgttgacagcgaagcttcgtggaacagcgtgaccgtcgttactcactggatttgccggtgaatttgatgagtcaaaaatataactagcagctggtcaaagtaaccactctgaataagacacgtgtcagaaactttgttgaccattctgactaaagaaaccttgtaaccaaaaacatccacatttttacatgctctgtcatatttcaactgtatactaaagttgaaatatgactatggtaacttatgtttttttagttgaaaactaaggtaaactattctatgccagcaggtaaaagatgtggatgaccaactactgctggcataatttattctatgactaaggtaaaactaaaagttaatatcactcgaaatatttacaaaagtattagataaagtactaaaaattttaagttagaaatgatgaaattaaaagatatatgtggcttatttaggaaaatagatacttttaatatgatggttgggtagttttattattgtttgggattgaaaaaaactatgaaagtgtctccaagtacagtaatatttaacaactaactaggaaggtgtacattgttcagtattcatcattctaattaatacaaataattttaaaaatttggggtcgtcaattgctcaaagatattcattattttataattttctacattttatcaaaaacagaattgtgtaaatgttgtgtcattatgtgtcgacttggatgtatgcattacataattttattttatatatgtttttaattgttagagcatttattcgaaaattataaatattgaattttaatcctcagtcacttaataaaaacattattttaggactaaaaaataat

SEQ ID NO: 53 - DNA, 1000 bp, Oryza sativa
caacgacggcttgcaggaatttttaaaaaactataaaaaaaatcatatcaataatacggatcttaccggtgtagtgagatgacaaagaagagaagcaatgggcaggtgagcgtgcgcaaacaaatgagataggaggcagttgccacaggagggcatgccgagggtggtaaagtaaataaaaaaataattataagagttcaagtagaattacaatttataaatgaaagaaatatcacaataagaaatatttatttttgaaaaaaatagtccatacagaccacaacatgacaaattataataaaaaaacaagagaatagacccataaaaaattagagtggtgtaggtagatgggacatctaaaaactataaacaaaaccttaaatagaatatcaatgataattaagaggagggacaacgagccggtcgttaagcagcacgatctcgacgattggagggatttctagaaagtaaaaaaaaactctcaattataatcatgttcgattttcaaatctcaacgataataaaaatgggaagcaatggacgggccaaagaggagtatagtggcggcgtttagcgagacttataaaaattataaaaatgaaacccaacaatacaatgaactctaaaaccacaaggtcaaatttgtagaggttccaggaaggatgaatgaaagcattggtagatcgagcaagtaaataaagcgatgataaagaaataatgcgtagtgattagcatgactattaaaagcaccgggatgataaagtcggtttctaacatatagttatttaacaaattttaagtaaaatcatatgtaaaaaatagataattttgtatgggtgctagcccgcgcaattgcgcgggccacctagctagtttttttaaaaatgtaaatataaaaaattcgaccaccacgcatcgcctgctctgccgcggcgacgcgagccacaaagccgtcgaccaccgcaacaacaaaatatcctcctcccgacgcaaaccggtt

SEQ ID NO: 54 - DNA, 1000 bp, Solanum lycopersicum
atgtttaatttatgggtaatgtagaagtgtatttaaaaaaaaaaaattgataaatatgtttatattatatgtgtaatgtgtgttaatattttcggtgatggaataatatatgataaatcatttagactcatgaagctcttcttaaatataatgaaaagacttccaatgtaaaaaattataatcggaagcggagccaatatatatttaggggttcatttgaattctctttagcgaaaaatatagtactatttatatatgatcagttatttttttttatgcatatgtagtagatattaaatctccttcgattatttcgtgtgtttacttcttgagattttaaattccctattcaaaaatcctagcctcgccattgtccgtaacaaagagatactaaatcgtatcttgtactccctgtgtcccaatttatgcgacttacgttgctttttagtcagtccaaaaataatgacacaattctatattaagtaacaatttaactataaaacgtcgattttatccttaatgaaacgatttaccaccacacaaatttctcattttagactgcaagttttttaaaaattttcatttctttcttaaaactctgtgccgaataaaactactttacgtaaaatagaaaggaggaaatatttatttacacatcataaaaagtctcgaggaaaatcaaaaaaacgtcacaacaaacataatattttcattgaaaaaatcgtttcatacctatttcttttgttgtctctttttcatccagtgttcagtactcactataaacactgaccaatataaaactattcgcgctccaaaataccacattaaataaaagcaacttcatacataaaactcgaactcataatctcccgttataaaaggataccacaactttttagtgctctttttcaataataactttttttttataaaaaaaaactaactgccagagtggaatttccaactgtatctatttgatgaaaatagcagaaaactggtt

SEQ ID NO: 55 - DNA, 26 bp, Artificial sequence
  Synthetic primer
cgcaggtatcacgaggcaagtgctaa

SEQ ID NO: 56 - DNA, 26 bp, Artificial sequence
  Synthetic primer
gtgtactcatgtgcatctgacttgac